European Patent Application EP 4 265 713 A1, published October 25, 2023. Title: Genetically modified methylotrophic bacteria producing lactate. Applicant: Acies Bio d.o.o. The sequence listing filed with the application follows.

SEQUENCE LISTING (181 sequences)

SEQ ID NO: 1 - protein, 333 aa, Methylobacillus flagellatus
MRIVFFSTQVYDRESFLALPRLQNAEFIFQQPKLTLDTAVLATGAEVVCAFINDDLSAPVLERLAANGTKLIALRSAGYNHIDLEAAQRLNLAVVRVPAYSPHAIAEHTVALILALNRHLTRAYNRTREGDFSLRGLTGFDLVHKTVGIIGTGQIGAAFARIMAGFGCRILAYDPYPNPEVIALGASYLELDTLLAQSHIVSLHCPLSPATHHLINAGSLSRMQPGSMLINTSRGALVDTPAVIEALKSGHLGYLGLDVYEEEADLFFEDLSDFPLQDDVLARLLTFPNVIITAHQAFLTREALNAIASTTLDNISAWAAGHPQNLVRLETGS

SEQ ID NO: 2 - protein, 333 aa, Methylobacillus sp
MRIVFFSTQVYDRESFLALPRLQNAEFIFQQPKLTLDTAVLATGAEVVCAFINDDLSAPVLERLAASGTKLIALRSAGYNHIDLEAAQRLNLAVVRVPAYSPHAIAEHTVALILALNRHLTRAYNRTREGDFSLRGLTGFDLVHKTVGIIGTGQIGAAFARIMAGFGCRILAYDPYPNPEVIALGASYLELDTLLAQSHIVSLHCPLSPATHHLINAGSLSRMQPGSMLINTSRGALVDTPAVIEALKSGHLGYLGLDVYEEEADLFFEDLSDFPLQDDVLARLLTFPNVIITAHQAFLTREALNAIASTTLDNISAWAAGHPQNLVRLETGS

SEQ ID NO: 3 - protein, 331 aa, Methylobacillus rhizosphaerae
MRIVFFSTQVYDKESFLAFPRLQNAEFIFQQPKLTVDTAVLADGAEVVCAFINDDLSAPVLEKLAANGTKLIALRSAGYNHIDLEAAQRLNLAVVRVPSYSPHAIAEHTVALILALNRHLTRAYNRTREGDFSLRGLTGFDLVNKTVGVVGTGQIGATFARIMAGFGCKILAYDPYPNPQVTALGASYLELDTLLAQSHIVSLHCPLSPETHHLINASSLSRMQQGSMLINTSRGALVDTPAVIEALKRGHLGYLGLDVYEEEADLFFEDLSDFPLQDDVLARLLTFPNVIITAHQAFLTREALDAIAGTTLANIDAWAAGRPQNLVRLET

SEQ ID NO: 4 - protein, 331 aa, Methylobacillus methanolivorans
MRIVFFSTQAYDRESFLAFPKPQNAEFIFQQPKLTTDTAVLAAGAEVVCAFINDDLSAPVLEKLASGGTKLIALRSAGYNHIDLEAAQKLGLAVARVPSYSPHAIAEHTVALILALNRHLTRAYNRTREGDFSLRGLTGFDLVNKTVGVIGTGQIGAAFARIMAGFGCKVLAYDPYPNPEVIALGACYLDLDTLLAQSHIVSLHCPLSPATHHLINANSLAHMRRGSMLINTSRGALVDTPAVIDALKSGHLGYLGLDVYEEEADLFFEDLSDFPLQDDVLARLLTFPNVIITAHQAFLTREALDAIASTTLSNIEQWATGTPQNLVRLEA

SEQ ID NO: 5 - protein, 331 aa, Methylobacillus arboreus
MRIVFFSTQVYDRESFLALPRSPNTEFVFQQPKLTADTAVLAAGAEVVCAFINDDLSAPVLETLAAGGTKLIALRSAGYNHIDLEAAHTLKLEVVRVPAYSPHAIAEHTVALILALNRHLTRAYNRTREGDFSLRGLTGFDLVNKTVGVIGTGQIGTAFARIMAGFGCKILAYDPYPNPEVEALGVRYLELDELLAQSQIVSLHCPLSPATYHLINESALNRMQRGSMLINTSRGALVDTPTVIDALKSGHLGYLGLDVYEEEADLFFEDLSDFPLQDDVLARLLTFPNVIITAHQAFLTHEALDAIASTTLDNIVAWAEGRPQNLVKLET

SEQ ID NO: 6 - protein, 331 aa, Methylobacillus caricis
MRIVFFSTQAYDRESFLEHDKPNDAEFVFQQPKLTLETAVLAAGAEVVCAFINDDLSAPVLEQLAANGTRLIALRSAGYNHIDLEAATRLGLAVARVPSYSPHAIAEHTVALILALNRHLTRAYNRTREGDFSLRGLTGFDLVNKTVGIIGTGQIGAAFAKIMAGFGCKLLAYDPYPNPKVVKLGAQYLELDELFGQAQIVSLHCPLSPSTYHLINASTLGRMQSGSMLINTSRGALVDTPAVIEALKSGHLGYLGLDVYEEEADLFFEDLSDFPLQDDVLARLLTFPNVIITAHQAFLTREALNAIASTTLANISAWAEGSPQNLVNIEG

SEQ ID NO: 7 - protein, 331 aa, Methylobacillus gramineus
MRIVFFSTQTYDRESFLGLDKPTGAEFVFQQPKLTVDTAVLAAGAEVVCAFINDDLSAPVLDQLAATGTRLIALRSAGYNHIDLEAAQRLGLVVTRVPSYSPNAIAEHTIALILALNRHLTRAYNRTREGDFNLRGLTGFDLANKTVGIIGTGQIGAAFARIMAGFGCKLLAYDPYPNPEVTALGAEYLPLDALFSRAQIVSLHCPLSPNTFHLINAETLNRMQRGSMLINTSRGALVDTPAVIEALKSGHLGYLGLDVYEEEADLFFEDLSDFPLQDDVLARLLTFPNVIITAHQAFLTREALHAIASTTLANISAWAAGSPCNLVKAEA

SEQ ID NO: 8 - protein, 330 aa, Methylobacillus glycogenes
MQIVFFSTQAYDRESFLSQPALSDCELVFQQPKLTVDTAVLAAGAEVVCAFINDDLSAAVLEKLAAGGTRLIALRSAGYNHIDLEAAKRLALAVVHVPSYSPHAIAEHTIALILALNRHLNRAYNRTREGDFSLRGLTGFDLVNKTVGIIGTGQIGAAFARIMAGFGCRLLAYDPYPNPEVIALGAEYLPLEQLFPQAHIVSLHCPLSPATHHLINPQTLALMQKGSMLINTSRGALVDTPAVIEALKTGHLGHLGLDVYEEEADLFFSDLSDYPLQDDVLARLLTFPNVIITAHQAFLTREALAGIASTTLLNVAAWRRGQPQNLVQPG

SEQ ID NO: 9 - protein, 329 aa, Escherichia coli
MKLAVYSTKQYDKKYLQQVNESFGFELEFFDFLLTEKTAKTANGCEAVCIFVNDDGSRPVLEELKKHGVKYIALRCAGFNNVDLDAAKELGLKVVRVPAYDPEAVAEHAIGMMMTLNRRIHRAYQRTRDANFSLEGLTGFTMYGKTAGVIGTGKIGVAMLRILKGFGMRLLAFDPYPSAAALELGVEYVDLPTLFSESDVISLHCPLTPENYHLLNEAAFEQMKNGVMIVNTSRGALIDSQAAIEALKNQKIGSLGMDVYENERDLFFEDKSNDVIQDDVFRRLSACHNVLFTGHQAFLTAEALTSISQTTLQNLSNLEKGETCPNELV

SEQ ID NO: 10 - protein, 335 aa, Fusobacterium nucleatum
MQKTKIIFFDIKDYDKEFFKKYGADYNFEMTFLKVRLTEETANLTKGYDVVCGFANDNINKETIDIMAENGIKLLAMRCAGFNNVSLKDVNERFKVVRVPAYSPHAIAEYTVGLILAVNRKINKAYVRTREGNFSINGLMGIDLYEKTAGIIGTGKIGQILIKILRGFDMKVIAYDLFPNQKVADELGFEYVSLDELYANSDIISLNCPLTKDTKYMINRRSMLKMKDGVILVNTGRGMLIDSADLVEALKDKKIGAVALDVYEEEENYFFEDKSTQVIEDDILGRLLSFYNVLITSHQAYFTKEAVGAITVTTLNNIKDFVEGRPLVNEVPQNQ

SEQ ID NO: 11 - protein, 329 aa, Pseudomonas aeruginosa
MRILFFSSQAYDSESFQASNHRHGFELHFQQAHLQADTAVLAQGFEVVCAFVNDDLSRPVLERLAAGGTRLVALRSAGYNHVDLAAAEALGLPVVHVPAYSPHAVAEHAVGLILTLNRRLHRAYNRTREGDFSLHGLTGFDLHGKRVGVIGTGQIGETFARIMAGFGCELLAYDPYPNPRIQALGGRYLALDALLAESDIVSLHCPLTADTRHLIDAQRLATMKPGAMLINTGRGALVNAAALIEALKSGQLGYLGLDVYEEEADIFFEDRSDQPLQDDVLARLLSFPNVVVTAHQAFLTREALAAIADTTLDNIAAWQDGTPRNRVRA

SEQ ID NO: 12 - protein, 334 aa, Luteitalea pratensis
MDIAVFDTRAYDRHAFDAANTRYGHELRFFEPRLSSRTATLASGVPVVCPFVNDRADAETIGALHRGGTRLLALRSAGFNHVDLDAAAAIGMRVVRVPEYSPYAVAELAMCLVLTLNRKVHRAYNRVREANFSLEGLVGFDLHGKTFGIIGTGRIGRVLARIAHGFGCRVLATDASPDEALQRELGVEYVEASTLYREADVISLHVPLTTETHHMIDKDAFAQMKAGVMLINTSRGALVDARALIQALKSRHVGAAGLDVYEEEGPLFFRDLSAQVLQDDVLARLLTFPNVLITSHQGFLTREALANIADTTLASVSAFARGEALVHEIGQRVP

SEQ ID NO: 13 - protein, 331 aa, Streptomyces rubrolavendulae
MDVLAFGVQTDEKPLLERAFAGHHGLHCLDVFLTEDTAPLAAGHEAVSTSVNADLGARVLRTLAAGGTRLVAQRSTGFNNIDLDVARELGMTVARVSYYSPYSVAEFAWTLAMAVNRRVVRAAHRTRDFDFRLDGLLGRDMRGRTVGVLGTGKIGEAFTRIAHGFGMRLLGWDLAENPACRELGMAYVGKEELLAASDLVSLHVPLTEKTWHLLDADALAAMKDDAILVNSSRGGLVDTDALVAALRAGRFAGVGLDVYEAEAGLFHVDRSLTGVDDDTLARLMTFPNVLVTSHQAFYTQEAVGEIVAATLRNVTDYAEGRRSENVLVPAG

SEQ ID NO: 14 - protein, 334 aa, Aquifex aeolicus
MNVLFTSVPQEDVPFYQEALKDLSLKIYTTDVSKVPENELKKAELISVFVYDKLTEELLSKMPRLKLIHTRSVGFDHIDLDYCKKKGILVTHIPAYSPESVAEHTFAMILTLVKRLKRIEDRVKKLNFSQDSEILARELNRLTLGVIGTGRIGSRVAMYGLAFGMKVLCYDVVKREDLKEKGCVYTSLDELLKESDVISLHVPYTKETHHMINEERISLMKDGVYLINTARGKVVDTDALYRAYQRGKFSGLGLDVFEDEEILILKKYTEGKATDKNLKILELACKDNVIITPHIAYYTDKSLERIREETVKVVKAFVKGDLEQIKGNFVVGPS

SEQ ID NO: 15 - protein, 310 aa, Armatimonas rosea
MKIIVTAAYSDLEEEYDHMVRLLPEHDVAPTLAPDAPVLCVTSRDLVTLELLDSLPGVRLIATRSTGFEHIDLAAARARGITVCNVPHYGDHTVAEFAFGLLLTLKRHLHTVLKDADAGRFPFGGLRGLDLFGLTLGVVGAGRIGRCAAKIGVGFGMTVLAHDIAPLPDEAERIGFTYVGLDELLTRADVLTLHTPLTPQTYHLIGAAELARLPRGAVLINTARGSVVALAAVLQALDSGQLAGAALDVLEDEERIAELAPPLLERYPNLLLTPHVAYHTVGSVGRIRQTTADNIRAFLNGAPQNTVPLP

SEQ ID NO: 16 - protein, 347 aa, Neosartorya fumigata
MKLAVFSAKSYDKLFLDSSLEKDYASFCEIVYHSFALSSETVSLAKGSDAVCAFVNDTLDAPVLKSLHRYGIRAILLRCAGFNNVDLQVAEELGFFVANVPSYSPEAVAEFAVALIQTLNRKTHRAYNRVREGNFNLEGFLGHTLHGKTVGIVGVGRIGLALAKIFHGFGCRLLASDPFGGEEFRKYGEFVELSELLAQSDVVSLHCPLTESTRHIINDETLAQMRKGALLVNTSRGGLINTKAAIRALKEGHLGGLALDVYEGEGSLFYNDHSTEIIHDDTLMRLMTFPNVLVCGHQAFFTQEALCEIAGVTLGNLQDFVLKRTCKNSLVREGHLLVRRDTEPVRL

SEQ ID NO: 17 - protein, 340 aa, Flavobacterium sp.
MTKINLLSHKISFFSTQPYDQTFFEKYNADFGFELEFFDIQLNEQTVTLVDNKAIVCVFVNDVVNAAVIKKLAEKEVKIIALRCAGFNNVDLEAAKKHGIQVCRVPAYSPEAVAEHAMTMILTLNRKTHKAYNRVREQNFSLHGLLGFDLHGKTIGIIGTGNIGKAFSKIAKGFGSTVVAYDVVKDSGMEADGVQYVALDTLIKKSDIISLHCPLNDETRHLINKKTLAQMKTNVMIINTSRGALINTSDVIKGLKSGKVGYLGIDVYEQEEKLFFRDLSDDIIQDDKIQRLMSFPNVLVTAHQAFFTNEALTQIALITLSNVKELALNGQTKDQLTQLV

SEQ ID NO: 18 - protein, 260 aa, Thanatephorus cucumeris
MRCAGYNNVDLKVAKELGILVVNVPAYSPEAVAEFAVGMLLTIVRKYHKAYNRVREGNFLLDGLTGFNLEGKTIGILGTGKIGLCTGRILSHGFRAKVIGYDPYPNPTAAEENGIKYVSLDELFKTSDVISLHCPLTPETKYIVNEEALKTTKPGLIIVNTSRGALINTSDLIHGLKSGHVGAVGMDVYERESKYFFRDSSNKIIQDDQLSRLVSFHNVFISGHQAFLTQEALSAIARVTVENLRLLEEGSPCSNIVTEG

SEQ ID NO: 19 - protein, 337 aa, Candidatus Heimdallarchaeota archaeon
MKIAFFEVKSWEIDYLTKLFRTEEDFDLTFTDQPLNQKNVENFTDINIASVFIYSTINKSVLKSLNNLKFIATRSTGFDHIDLTECDNKNILISNVPYYGENTIAEHTFGLILALSRNIHKSYVRTQRNDYSIEGLKGFDLQGRTLGIIGLGRIGMHVARIARGFGMKVLAYDIKQDSFFSDLINFTYTSFEEVLKLSDIVTLHVPYNKHTHHLINKNTIKLFKKGAVLINTARGGVVETESLLEALENKTLSGIGLDVIEGEEYIKEEKQLLYDSEKIDIWKKIIQDHILLKKDNVVFTPHIAFYSQEALERILQTTKDNIKGFTSNRPQFIVTNK

SEQ ID NO: 20 - protein, 337 aa, Candidatus Hydrogenedentes bacterium
MSNIAIYDSKPYTRHSFEARNTGGLPITFFEHKLTGDTAGSAAGFDAVCIFVNDTVDAEVAMRLKELGVGLVALRCSGYNNVDLNACARHGISVVRVPGYSPPSVAEHSIALMLALNRHIMRAHARVREGNFSLNGLTGFEMRGKTAGIVGTGRIGTCAAEILSGFRCSILAYDPHPAEALSKNPRLRYTDMDTLLHQSDIISLYVPLLPTTRHLINDEAIRKMKRGVMLINTSRGALVDTAALIRGLKSGKVGSAGLDVYEEESDYFFEDRSEYIIADDLLARLLTFNNVLITSHQGFLTNEALDAIALTTFQNIQEYLEGKREKELSNGICPKCG

SEQ ID NO: 21 - protein, 274 aa, Microgenomates bacterium
MDIGFFEVNDWEVPIIQKHFPHAFISSEKLVAENAKKYKNLQVVSTFIYSQLNSSVLVQMPKLRCIATRSTGFDHVDAKYCARNNIVVCNVPRYGDRTVAEFTFALILSLTRRIYESVALTRLGSFDNHGLTGMDLEHKTIGIIGLGKIGQEVAKIARAFNMKILAFNRSHDDTLAAELGLEYVELNELLKRSDVVTLHLPLLPTTTHFINKNILTMKKGSYLINTARGGLVETQALIIGLHKGILAGVGLDVLEEESVLNEEAELISSEFRKK

SEQ ID NO: 22 - protein, 328 aa, Candidatus Nanohalobium constans
MTVEKVAWFDTENWEKEYLENKDFPFEIKFFEESLTKDTAAKTEGFDAVSVFVSSQVSSEVIEELDVDIIACRSTGFDHVDIETASEQGIKICNVPRYGANTVAEHAFGLILTLSRRIHEAISKVENGEFDHQGLKGFDLEGKTLGVVGTGSIGQKVIEMAHGFNMDVLASDPYPKEGLEEELGFMYVSMEDLIKKSDIITIHCPLTDENHHLFSEEQFKLMDETVLINTARGELVDTTALIRALENGNVSRAGLDVLEEECVIEEDIEILGDISDECDPQKIVEDHILMERDDVVVTPHNAFNSREALQRIEDKTLENIEKGRNTVN

SEQ ID NO: 23 - protein, 332 aa, Candidatus Peregrinibacteria bacterium
MKIAFLEVSKSDKIFLRRRLPDDELIFINENLNEENIKKIKDCEVLSVFIYSQVNKKNLDKLLKLKLITTRSTGFDHIDAQTCKNKGISICNVPFYGENTVAEHTFALILALSRNVHKSYLRTLRRDYSTTGLMGFDLKGKTLGVIGAGRIGLHVIRIAKGFGMNVLAFDLNRDKFISEILDFSYGTIEEVLKASDIITLHVPYNKYTHHLINKDNLRLVKKGAILINTARGGIIETQAIIEALDKGLLSGVGIDVLEGEEMVLEEKKLNFDEKNLESMSHLIQDHILLSRDNVVFTPHIGFYSKEALERILETTVESIEGFKKGNLVNSIS

SEQ ID NO: 24 - protein, 347 aa, Candidate division BRC1 bacterium
MTRKIAFFDAKPYDIKSFTEMNKDFGFDIAYFETHLNAQTASLSGDFDAVCAFVNDTIDKAVIDEIIKHGVKLIALRCAGYNNVDFKAAYKKIHIARVPAYSPYAVAEHAAALMFSLNRKTHRAFFRTRDGNFSLNGLLGFDMHGKTAGVIGTGKIGKCLIAILKGVGMKLLAYDPFPDEAFAADAGVQYVSLDEIYQQADIISLHCPLNKDTEYMINAQAISRMKNGVMIINTGRGKLIHTQALIDGLKSGKIGAAGLDVYEEESEYFFEDKSAQMITDDILARLLMFPNVLVTSHQAFFTQEALRNIAQTTLQNCQDFFEHEKLVNEICYKCGGPCTRKEKKLCF

SEQ ID NO: 25 - protein, 327 aa, Methanomethylophilus alvus
MKVFVYNYRRFDEEKYFQQYAEEFGFELGYTEESPTIDNCGLADGCDFISIITTPITPEMMDRFKEGGVRMISTRTIGYDHIDIAYAKRIGMTVTHITYDPEGVAEYTVMMMLMAIRKAKNILERGKDNDFTLDGLIGGELGDMSVGIIGTGRIGRSVLRDLSGFGCRLYYCNRSPSEEADRYAERVDMDELLGMCDVVSLHLELNKDTFHIMGPEAISKMKKGALIVNTARGPLIDTDALAAGLDSGQVGGAALDVIEDEFGLYYYDCSGRELDNKALKVLRGRPNVLITQHMAFYYENAIRDMVYNSLYGMKMLADGKEIPYRLA

SEQ ID NO: 26 - protein, 339 aa, Candidatus Wolfebacteria bacterium
MKIAFFQIEDWEIEHIKEQLAGHELFFSKEKLSAEALPEQRDFDIVSVFVGSKIDQAVLAALPNLKLVTTRSTGFDHVDLPMAQSMNIATGYVPGYGDNTVAEFAFGLILALSRKIYDSVDRLRETGVYSYVGLRGFDLQGKTIGVMGTGRIGQHVIRIAKGFGMQVIAFDAFPKAELATELGFEYVGLDDLLGRSDVITIHVPYLPSTHHLINMDSLTKIKKGALLINTARGAVVETDALVKGLADGILGGAGLDVLEEEGVLADEKTLVLYGHPEEHNLKTVLENHVLIDMPNVLVTPHNAFNTQEALQRILDTDICNIQEFLGKGIAKCPIPAPKA

SEQ ID NO: 27 - protein, 202 aa, Candidatus Anoxychlamydiales bacterium
MKIAIFGSQEYDIESLNEANKKYSNDLTFFKAYLNEKTASLAKNFDAVCLFVQDTANKAVIDILAKQGVKTIALRCAGFNNVDLDSAKTNNISVVNVPAYSPHAVAEHAVGLILSLNRKIHHAYTRIRDGNFSLKGFLGFDLYGKTVGVIGTGKIGQETAKIFKLGFGCKVIASDPYPNKTLEKECQSPLPKGRGLNREDQG

SEQ ID NO: 28 - protein, 453 aa, Monoraphidium neglectum
MRAPAQQPRAAGAARGPATAPRAPALRGATWRGACRVATQVDAVEAPRPADPVEAPKPASDPELAAKRSAFKIMTFSAQPYVNKYFLEPLQAAGFDNIKGTEASAGTGAPRACGRACTQRQRQPPPAEPGHASARLGIDTVKIASGYDAICLFVNDLCDAEVINALAEGGVKFIAMRCAGYDRVDVAAANAAGIKVVRVPTYSPTSVAEHAVALLFAIDRHIVGAINRVTQGNYSLSGLVGRQLGGKTIGILGTGAIGAEAARIFKGIGMKVLAYDIRPNPAVEALGIPYLPWEEILPQADVISLHMPLLPSTYHFIDEAKVAMMKPGVVLLNVSRGGLIDTPALIYGVRSGHIGGAGLDVYEKEGERPCPRAARGVALRDLTDLQPRDRMVFWDRRLIELIALPQVLVTPHTAFLTAEALVNIADTTVQNIDQFMLGKPLGNEVKPPPPAKS

SEQ ID NO: 29 - protein, 482 aa, Rattus norvegicus
MLLRVATQRLSPWRGYCSRGSQGGLSQDFVEALKAVVGSPHVSTASAVRQHHGHDESMHRCRPPDAVVWPQNVDQVSRLASLCYNQGVPIIPFGTGTGVEGGVCAVQGGVCISLTHMDQIMELNTEDFSVVVEPGVTRKALNTHLRNSGLWFPVDPGADASLCGMAATGASGTNAVRYGTMRDNVINLEVVLPDGRLLHTAGRGRHYRKSAAGYNLTGLFVGSEGTLGIITSATLRLHPAPEATVAATCAFPSVQAAVDSTVQILQAAVPVARIEFLDEVMMDACNRHSKLNCPVAPTLFLEFHGSQQALAEQLQRTEAITQDNGGSHFSWAKEAEKRNELWAARHNAWYAALALRPGSKAYSTDVCVPISRLPEILVETKEELKASKLTGVIVGHVGDGNFHCILLVNPDDVEEQRRVKAFAENLGRRALALHGTCTGEHGIGLGKRQLLQEEVGPVGVETMRQLKDTLDPRGLMNPGKVL

SEQ ID NO: 30 - protein, 323 aa, Desulfurispira natronophila
MTDVFFYEAFAEEAEQLQRFLPNSVSAGFTDRTIQESGDAHPPARVISVRTQSAIPPSWSPHIEAILTRSTGFDHIQRYFWETGQKIAAGYLPLYCNRSVAEQAMLLWMALLRQLPRQMEQFGSFHRDGITGGEAQGRTLMVAGVGNIGHEICRIGSGLGMTVLGVDIDERHDDVLYVSPHEAIQQAHVIVCSMCLTNENRHYFHYDMLRQARPGAVFVNIARGELSPPADLMRALDESILAGVALDVFDEEKELATALRQGSLPVQPTVCQTLELARRSNVIMTPHNAFNTVESVERKSRQSLEQLQHFFATGEFLWPIGRN

SEQ ID NO: 31 - protein, 473 aa, Aeropyrum pernix
MARIAEELEKIFGPEKVVSDPHIVRLYSREPSGLEGRAEAVVFPESAQDVSRLVRYAYSREVYIYPQGSSTDLAGGAFPERPGVVVSMERMRRVREVSVLDSVAVVEPGVRLWDLNVELSKYRYMFPIDPGSVKVATVGGAINTGAGGMRGARYGTMRDWVLGLEIVLPDEEGTILRVGCRTLKCRQGYDLARLIVGSEGTLAIVTEAILKITPMPENVVVVLAFFPTLRQLVDAVIEVKSRAIDTLLMEFMDVDSARLAAETLGAAIRPDGHMLLVGVPVNREASTRVLEEMVSIAKAAGAASVYTAKSMEEAEEKKLLEIRRSLFATQALLTQKQFKGRKVMMLMEDIAVPPSKLLDAVERLKELEAKYGFKTVLGGHIGDGNLHPTISYPVDDEKAKEAALKWYYDVMRMAIELGGTVSAEHGIGVLKKEALRLELERMGSVKALEIMAGIKRVFDPKGILNPGKVVAAE

SEQ ID NO: 32 - protein, 333 aa, Synechocystis sp.
MKIAFFSSKAYDRQFFERANHHHGREMLFFDAQLNLDTAILAEDCPVVCLFVNDQAPAPVLEKLAAQGTTLIALRSAGYNNVDLKTAAALGLKVVHVPSYSPHAVAEHTVGLILALNRKLYRAYNRVRDDNFSLEGLLGFDLHGSTVGIIGTGKIGLAFAKIMNGFGCHLLGYDAFPNENFTAIGQAIYVPLNELLAQSDIISLHCPLLPETHYLINSSTIARMKPGVMLINTSRGHLIDTQAVIQGIKSHQIGFLGIDVYEEEEALFFTDHSDTIIQDDTFQLLQSFPNVMITAHQGFFTHNALETIAETTLANIAEFEQNQPLTYEVICPH

SEQ ID NO: 33 - protein, 349 aa, Elusimicrobia bacterium
MERIKLAFFDAKPYDIEFFNIENAKYGYHIKYFLNRLNSDTVAMSQGFNAVCIFVNDNVTKDVVKILLKNKIKIIALRCAGYNNVDLSSVYNKIHVVRVPDYSPYAVAEHTVGIMLSLNRKIHKAYYRTRDNNFNINGLLGFDMNGKTAGIIGTGKIGKVLIKILKGFNVKILAYDPYPDKDFAEKMEISYVPLDKLYRSSDIISLHCPLTKDTFHLIDHSAISKMKTGVMVINTGRGRLIDTKALIEALKHGKIGSAGLDVYEEESEYFFEDFSDKILPDDALARLLSFNNVLITSHQAFFTKEALTNIARTTLGNIFAYSKGEKLANEVCYKCDKRSCCSGKSGKCF

SEQ ID NO: 34 - protein, 310 aa, Methanoculleus bourgensis
MVVKLVFFDLDEHEQDVVRDAFASESGYEVDLHSDALTRQNVSLARDADGIAVFVTSHVTREVLDRLPNLKVIAAMSTGFDHIDVDTCRERKIAVCNVPLYGDTTVAEFAFGLILALARKFRPTFARTARGDFSRTGLQGMDLAGKTLGLIGTGRIGSHLARLAHAAGMNVVAYDLHPNLALTKDYGVRYLDLDDLLREADVISLHVPYTKATHHLINADRLRLVKDTALLVNTSRAGVVDTQAVAAALREGRLGGGRTRYLRGGADLDRGGVFWGRRALGGRTQGCARELRHPAIGPGNTLAAQRLQYP

SEQ ID NO: 35 - protein, 340 aa, Dictyostelium discoideum
MKITLFSSKPYWVKWFNELNKFSYEINYVTSACDIKSVNEAKGSEAVCCFVNDDLSKEVIETLHSNGTKVILMRCAGFNKVDLDTANKLGIPVLRVPAYSPNAVSEYALSLIMALNRKTHKAHDRVRDANFEINGMEGFNMVSKVYGIVGTGNIGEQLCRVLKLGFGAKVIAYDIIENKAVTDIGIEYVKTLDEIWKQCDVISLHTPLNSQTKYMVNSESIEKMRDGVMIINVSRGALVNASDAIVGLKSGKISSLGMDVYENETDYFYQDHNGSIIKDDNLSLLISYPNVMITSHQAWYTKEAISCICGTSLQNFVDFRSNQIKKSNLVNNPISSQPTQ

SEQ ID NO: 36 - protein, 333 aa, Lactobacillus delbrueckii subsp. bulgaricus
MTKIFAYAIREDEKPFLKEWEDAHKDVEVEYTDKLLTPETVALAKGADGVVVYQQLDYTAETLQALADNGITKMSLRNVGVDNIDMAKAKELGFQITNVPVYSPNAIAEHAAIQAARILRQDKAMDEKVARHDLRWAPTIGREVRDQVVGVIGTGHIGQVFMQIMEGFGAKVIAYDIFRNPELEKKGYYVDSLDDLYKQADVISLHVPDVPANVHMINDESIAKMKQDVVIVNVSRGPLVDTDAVIRGLDSGKIFGYAMDVYEGEVGIFNEDWEGKEFPDARLADLIARPNVLVTPHTAFYTTHAVRNMVVKAFDNNLELVEGKEAETPVKVG

SEQ ID NO: 37 - protein, 332 aa, Fusobacterium gonidiaformans
MIKMRVLFFDAKSYDKENFDAYKEKYGFDIKYLKVKLNEETVDFVKGYEIISIFVNDTVNPPVIDKLIEYGVKLIVLRCAGYNNVDVNYINGRIKLVRVPAYSPYSVAEYTASMVMTLNRKIHKAYVRTREGNFSINGLMGFDLHKKTVGVIGAGRIARIFIKIMRGFDARVIAYDPYPNESFARDLGYEYVDLDTLYRESDIISLHCPLTRENTYLINRESMKKMKDGVMIVNTGRGRLIDTIDLIEALKDKKVGAAALDVYEEEAGYFFEDMSSSIIEDDILGRLLSFNNVLLTSHQAYFTKEAFRDITLTTLENIQSFLQGKELENEIK

SEQ ID NO: 38 - protein, 360 aa, Kiritimatiella glycovorans
MSAPSILFFDAKSYDREFFQAANGNFGYELTFLGHRLTGESARLAEGHDAVCAFVNDRLSPEVADTLADSGIGLVALRCAGYNNVDLRSFFGRIHVVRVPAYSPHAVAEHTLALILSLNRKTHRAYYRTRDGNFAIEGLLGFDMAGKTAGVVGTGSIGRCAAQLLRGFGMEVLAFDVNPDLEWAERSGVTYVDMGELYRRSHLITLHCPLTSDNHHMINADTIGQMRDGVMIINTGRGGLIDAPALTEALKDRKVGAAGLDVYEEEDQYFFEDFSVRGLDDDVLARLLTFPNVLITSHQAFFTREALTNIADTTLGNIRDYFEGRPLENEICYRCCDEGCRKEEKGRCFESGPESAPPSE

SEQ ID NO: 39 - protein, 363 aa, Lentisphaerae bacterium
MQDKIRIAFFDTKPYDRLSFDAIKERYHVEIVYFETRLTPASAKLAEGFDAVCAFVNDDLCAETIHTLEALNVRLIAMRCAGFNNVDLAAACHRMKVVRVPKYSPYAVAEYTIGLLLCLNRHLHRAFCRIRENNFSINGFMGFDLHGKTFGIIGTGKIGLTFAQILGGFGVRILASDPFPNEKAAAELKMEYVPFETLYRESDVISLHCPLTPENHHMICSDTIGQMKTGVFILNTSRGKLIDTSDLIEALKSGKVGGAGLDVYEEEADYFFEDRSDRWINDDVLARLMTFPNVLITSHQAFFTREAVNNIAEITMDNIRDFQEGRELVNDVCFHCDGTRPCCHAKENTATSNPETSGSSASR

SEQ ID NO: 40 - protein, 332 aa, Stieleria varia
MKIAVFSTKPYDESFLRAASENHSHTLTFLEPRLTAKTAALANGFDAVCAFVNDQLDSDVIHTLSDHGVRAIALRCAGFNNVDLAAASECGVTVVRVPAYSPHAVAEHTAALVLALNRKIHRAYTRVRDGNFALGGLLGFDLNGRRVGVVGTGKIGEIFAKIMSGFGCKLLGFDVQQNPECERLGMQYVSLDELFAESDVISLHCPLTPQTHHLIDAAAIQKMKPGVMIVNTSRGAVIDTGAVINGLKSGKIGHLGIDVYEEEADLFFEDLSSQVIPDDMLSRLLTFPNVIVTGHQGFFTEEALSCIAETTLQNLTDLESTGNCPNAVTTTG

SEQ ID NO: 41 - protein, 329 aa, Escherichia coli; identical to SEQ ID NO: 9

SEQ ID NO: 42 - protein, 340 aa, Galdieria sulphuraria
MSKSLFRVVVFSTKNYDQIGLTEALGRSSDAAPISFRFLSSRLSASTAELAKDAEAVCVFVNDTVNSEVLKILHDKGIQLIALRCAGFNNVDLKAASELGISVVRVPAYSPNAVGEFVAAQLLTLARKIHKAYNRVRENNFDLQGLVGIEIRGKKAGIVGTGKIGVATAKVLKGLGLELFGFDVFHNQEFIDLGGQYLSLDELLSQSDIVSLHCPLNESTKYLIRSETIAKMKSGAYLINTSRGALLDTQAVLDALYSGHIGALAIDVYEGEGDLFFEDRSGAIVHDPILAKLQALPNVLVTGHQAFLTDVALRNICNITIDNLSNFYYQRPLKNKVDPK

SEQ ID NO: 43 - protein, 331 aa, Treponema pallidum
MRCVVFNLREEEAPYVEKWKQSHPGVVVDTYEEPLTAKNKELLKGYEGLVVMQFLAMEDEVYDYMGACKLKVLSTRTAGFDMYNATLLKKHGIRLTNVPSYSPNAIGEYALAAALQLTRHAREIETFVRKRDFRWQKPILSKELRCSRVGILGTGRIGQAAARLFKGVGAQVVGFDPYPNDAAKEWLTYVSMDELLSTSDVISLHMPATKDSHHLINAKTIAQMKDGVYLVNTARGAVIDSQALLDSLDKGKIAGAALDAYEFEGPYIPKDNGNNPITDTVYARLVAHERIIYTPHIAFYTETAIENMVFNSLDACTTVLRGEPCAAEIKL

SEQ ID NO: 44 - protein, 313 aa, Vitis vinifera
MESIGVLLTCPMNPYLEQELDKRFKLFRFWDFPSANDLFREHSNSIRAVVGNSFIGADAQMIEALPKMEIVSSFSVGLDKIDLVRCKEKGIRVTNTPDVLTEDVADLALALILATLRRICESDRYVRSGSWKKGDFKLTTKFTGKSVGIIGLGRIGSAIAKRAEGFSCPISYHSRTEKPGTNYKYYPSVVELASNCQILVVACALTPETRHIINREVINALGPKGVVINIGRGLHVDEPELVSALVEGRLGGAGLDVFENEPNVPEELLAMDNVVLLPHVGSGTVETRKDMADLVLGNLEAHFLNKPLLTPVV

SEQ ID NO: 45 - protein, 345 aa, Mycoplasmopsis maculosa
MKIAFFDAKSYDKKYFDLVNKGEHEIVYFEENLNINNVNLAEGFDAVCCFVNTFGDKYILELLSQLGVKVWLQRSMGYNKVDLFAAKELGINVFRVPNYSAESVSEFAVTLLMTLNRNVNKAIERVKQYNFNLDGLDGKSIIGSTVGVIGAGKIGQGFIRALKGMGARVLVYDAYSEQNLPNLAIELGFEYAPFTKILRESDFISLHAPSLPSTKYIIDKDAVNLMKKDVVIVNTARGDLVDIKAILYGLENNIIRGFGADVLDREEGRFYEDISKNAFEYKQQDPEWQKLIEDNRVIITSHQAFLTDVALGQIAKITLSNASNAENGNFEGALTLLDDGRVLNG

SEQ ID NO: 46 - protein, 349 aa, Thermodesulfobacterium geofontis
MIWKIGFFEIEKDWEKNLYLKKFKETLKEKIEDTEIYFYEETLNENNVKRFRDLNIIIIHAESKINSTVVENLVDTKLLITRTTGTDHIDVLSCEKKGILVANCPVYASTTVAEHTVALMFALARKLKIAIDKNKKLDFSRDELMGIDLFGKTVGIIGTGRIGSEIARIVYGIGMKILATDVSPNNELVEKYKVKYVDLETLLKESDIIIVMVPYYSQTHHLINRENIKLVKEDAIFINTARGPIVDIEALIWALKNNKLQGGIAMDVFEGERVLMEFQNNLINGAFTAEEYERALKTLSLLNYSNIIFTPHIAYYTKEAMERVIDWVVENISRFLVCQVLPFQYKFYF

SEQ ID NO: 47 - protein, 343 aa, Defluviitoga tunisiensis
MSKNYKIAIVNSSTFGVYFPDLIQRLKKIGDIERIEVDPNINGKNLAKKLKGFTFVISSVTPTFSEEFFRYNKDVKLIARHGIGYNNVDIKAATENEVMVTRVYGVHERDAVAEIAVSLMLICLRGIIPAYQAVLQNKWHERKNFVGKELSKITVGIIGYGNIGSRVGEIVKEGFKSEVIAYDPYIADKVIEKTGVQPVEFDELFKKSDVISLNASLNEGNYHFINKKAFQKMKDGVVIVNTARGELINLPDFVEALETGKVFAAGLDVLETEPIEPDNPLLKFPNVYIVPHIGGYGTYSLRKMDEKMVEDIEKLVNGEIPDQIVNPEVISKILETFQGKNNR

SEQ ID NO: 48 - protein, 329 aa, Lacunisphaera limnophila
MRVVVFSTKPHDRQFLDAANAGRHDLVYLEARLLPETATLAAGAQAACLFVHDHADAAVLATFAGLGVKHLALRCAGFNNVDLAAAARLGITVARVPAYSPHGVAEHAVALFLTLNRRIHRAYNRVRDGNFSLDGLLGFDVHGKTVGVIGTGKIGLCFAQIMRGFGCRVLAFDVTRQPAAEALGVEYTTLERLYAESDLISLHCPLTPQTQHLIGAGALAQMRDGVYIVNTSRGPLIDTGAVIDALKSGRLGALALDVYEEEEGVFYEDLSGDILADDQLARLLSFPNVLVTSHQAFFTREAVTAIAATTLGNLDDFAAGRPCPHALKA

SEQ ID NO: 49 - protein, 396 aa, Escherichia coli [sequence omitted]

SEQ ID NO: 50 - protein, 320 aa, Pedicoccus sp
MSKIQNHQKVVLVGDGAVGSSYAFAMAQQGIAEEFVIVDVVKDRTVGDALDLEDATPFTAPKNIYSGEYSDCKDADLVVITAGAPQKPGETRLDLVNKNLNILSTIVKPVVDSGFDGIFLVAANPVDILTYATWKFSGFPKEKVIGSGISLDSARLRVALGKKFNVSPDSVDAYIMGEHGDSEFAAYSTASIGTKPLLDIAKEEGVSTDELAEIEDSVRNKAYEIINKKGATFYGVGTALMRISKAILRDENAVLPVGAYMDGEYGLNDIYIGTPAVINGQGLNRVIESPLSDDEMKKMTDSATTLKKVLTDGLKALEEK

SEQ ID NO: 51 - protein, 316 aa, Acidobacteria bacterium
MKAGVVGCGFVGSTAAYTMALGGVASELVLVDLVPALAKAHAEDILHATPFAAPVRVVGGDYPQLEGAHVVILACGVGQKPGETRLQLLERNAKVFEQVVPQVLKAAPSAILLVASNPVDIITRMVTHISGLSPARVIGSGTILDTARFRTLLSEYLGVAPQSVHAYVLGEHGDSEVLAWSSAKVGGISLEIFAAQRGVSIDDTVRARIDDGVRRAAYRIIEGKKATYFGIGAGLTRIVEAIRDDERVVLTVSICQDGLEGLEEVGLSLPRVVGRPGVIATLHPPLSPEEQDALCHSARVLQQAASELGFLERARA

SEQ ID NO: 52 - protein, 320 aa, Bifidobacterium longum subsp. longum
MAETTVKPTKLAVIGAGAVGSTLAFAAAQRGIAREIVLEDIAKERVEAEVLDMQHGSSFYPTVSIDGSDDPEICRDADMVVITAGPRQKPGQSRLELVGATVNILKAIMPNLVKVAPNAIYMLITNPVDIATHVAQKLTGLPENQIFGSGTNLDSARLRFLIAQQTGVNVKNVHAYIAGEHGDSEVPLWESATIGGVPMCDWTPLPGHDPLDADKREEIHQEVKNAAYKIINGKGATNYAIGMSGVDIIEAVLHDTNRILPVSSMLKDFHGISDICMSVPTLLNRQGVNNTINTPVSDKELAALKRSAETLKETAAQFGF

SEQ ID NO: 53 - protein, 334 aa, Helobdella robusta
MTSTTCVKELFTHIIDEERHTSVKVTVVGTGQVGMASAFAMLTQGVISELALVDMVADKLKGEMLDLQHGQAFLRTVKVQASTDYSVTAGSKICVVTAGARQNLGETRLQLVQKNVAIFKHIIPNLIKYSPNCILIIVSNPVDILTYVAWKISGLPRNQVIGSGTMLDSSRFRFILSERIGIAPKSVHGYIIGEHGDSSVAVWSSVNIAGTRLKDIHPHTGDPDDPENWNEIHKEVVNSAYEIIKLKGYTSWAIGVMISTLCNAILKNQKVIYSLSTLAKGYHGIEEEVFLSLPCVVGEKGVGAVFDQKLLPNEMEKVKASAKTLHDVIKSLEL

SEQ ID NO: 54 - protein, 316 aa, Plasmodium berghei
MAPKAKIVLVGSGMIGGVMATLIVQKNLGDVVMFDIVKNMPHGKALDTSHTNVMAYSNCKVSGSNTYDDLKDADVVIVTAGFTKAPGKSDKEWNRDDLLPLNNKIMIEIGGHIKNNCPNAFIIVVTNPVDVMVQLLHQHSGVPKNKIVGLGGVLDTSRLKYYISQKLNVCPRDVNAHIVGAHGNKMVLLKRYITVGGIPLQEFINNKKITDQELDAIFDRTINTALEIVNLHASPYVAPAAAIIEMAESYIRDLRKVLICSTLLEGQYGHKDIFAGTPLVIGGNGVEQVIELQLNADEKKKFDEAVAETSRMKALI

SEQ ID NO: 55 - protein, 308 aa, Armatimonadetes bacterium
MKVGIIGGGGRVGSNAAYALQLMGAVSEVVLLDVNREAAEGEALDLRHGAALSQPIRFRAGDYADLEGAEMVIITAGLRRRPDESRLELINRNVGLFRDILSQLRQVSLHPNVIFLVVSNPVDILTYLAVRESGLPAERVIGLGTVLDTCRFRSYLAEYFNVAATDVDALILGEHGDSMVPIWSCATIAGVPLKDYPGYSKEAMEQIFQQTRNAGAEAIRLKGGAGYAVGVSITQVVNAVALNQNAILPVSTLQTGALGIQDVCFSLPTRVGRNGVAGIIEIGVSNEERDALQNSAKVLKETLQKVIG

SEQ ID NO: 56 - protein, 250 aa, Spodoptera frugiperda
YSITADSQICVIAAGVRQMEGEDRRNLVQRNVEVLKGIVPKLLKYSPNAILLIASNPVDVLTYVTWKISGLPKHRVIGSGTNLDSARFRYLLSQKLNIAPTSCHAYIIGEHGDSSVPVWSSVNIAGVRLRDLNKNIGLDSDEENWKETHTQVVQSAYEVIKLKGYTSWAIGLSLTQLVKAILTNAASVHAVTTCVEGEHGITDNVFLSLPCVLGRNGVLDVIRQPLTDVEREQVFKSATLMAELQAKIKF

SEQ ID NO: 57 - protein, 318 aa, Lachancea dasiensis
MSEVQPATTPVKVVIIGVGSVGSATAYTLLLSKIVSEIVLIDVNKDKAEGESMDLNHAASSTTKSRAGDFPDCAGAAIVIVTCGINQKNGQTRMDLAAKNAAIMQEIVPNVAQHAPDSIILIATNPVDVLTYVSYKASGFPSSRVFGSGTVLDTARFKYILGEHFQIPSESVDACVIGEHGDSGVPVWSLTNIDGMKLREYCEARNHNYDEEVFHKIFEQTRNAAYDIIKRKGYTSYGIAAGLLRIVKAILGDTNAVLTVSTVGDYYGVEDIAISVPTRLDKDGVHPASEISLNQKELGLMKKSADQIKSALVALTQK

SEQ ID NO: 58 - protein, 327 aa, Atribacter laminatus
MNQKKQKISLVGVGRVGSTLALTILMKGLAQELVLVGENNHRAQGEAYDLIHASSFAHPIEIYAGPIEATSHSDIIVVSASVPMTNMKNRLDLGVGNAALFRNLIPQLSQLSPEAIFIIITNPVDIMTYYTIRLSNFPPSRVMGTGTLIDSGRFRSLLGLYSGIHSEDIHAYILGEHGDSEFPVLSLADFGGMGMEHSLPVCRKTCPLKNLTEVFEEAKDGGMLVYRHKGYTNHAIALATSTLIEAIFNDSGRILPVSTLIEGYLGVTDVCLSMPVVLGREGILKIIELNMNEKEQAAFRSSAAVLKKATQEMGIEKNMSEQRKPTE

SEQ ID NO: 59 - protein, 317 aa, Bacteroidetes bacterium
MTSNQGKRKVGVVGTGLVGSSLVYALMIRELATEIVLVDIDREKATGEMMDFNHGLSFSKPVKITAGNYADLKEAQVVVIAAGASQKPGETRLDLLARNVNIFRTIVPEVVQHNPTGIILIATNPVDILTHISLKESQLTAGKVIGSGTILDTSRFRFLLGQHYEVDARSVHAYIVGEHGDSEIPVWSLANIGGVRLQEFAPLKNKRYDQIEMDNLFAGVRDAAYEIIKRKGATYYAIGLGLVSIVETILGNYRSVLSVSTLMTGQYGVSDMCLSLPCVVGANGIEEILTLNLSPGEEKGFRLSAEKLKATLQSLGG

SEQ ID NO: 60 - protein, 328 aa, Rhodohalobacter barkolensis
MKKQEDRNHQKGSSAWKSRKVAIVGAGAVGATFAYAMAQNGAADEICLIDLNNELCKGQVLDLSHGLPFYPTINIYAGSEKDYADADVIVITAGAAQKKGETRLDLLKKNSAIIEGIVDQITAQDSKATIVVVTNPVDILTKIALERSGWDRSRVIGSGTVLDSSRFKYLLSEFFNVYVGSIHAYILGEHGDSEFAAWSMANISGVQLDEYSKQLGIDNWPEKKKEIELEVRDSAYHIIDYKGATNFGVGLALVQIVGAILKNQRRVLTVSYHLEGEYGISDICLATPCLISQNGVASIIGTELTKEEQEKLVNSANILKREYSELKR

SEQ ID NO: 61 - protein, 287 aa, Piloderma croceum
LLLRPIASDILLVDTDDLRLRAQVQDLSDAAFLSNTKIRPSTPVEAGQCNIIVITAGAKSRDGKSRRNLIDRNYLVLDNVIREMSPIRKDAVLLLVSNPVDVLAYFAQKMSGLPHAQVIGSGTFLDSVRLRSALADQVQVADTAVHAYVLGEHGDSQMAAWSTATVGGSPVQNFLSSTCPSLSDLANSAKTKAYSIIAAKGATAYGIASIVSSICESIILNQRHVRPVSHWIESLETYISLPAVLGHGGVQKTIEVPLDETEKELLQKSVEEIRSNIRTVEEGEQYQ

SEQ ID NO: 62 - protein, 316 aa, Caldithrix abyssi
MKIGIIGCGYVGSTVAYAVLFKKAATEIVLIDKNHQRAVAEAADISHAIPFSHAIDIYAGDYSDLKGAELVIIAAGVNQKPGETRLQLLGRNEAVLRQILPPLLENAPEAMILMTTNPVDVMTHLAAKLAEELGYNGHLVFGSGTTLDTARFRSLLSAKLGVAPQHVHGYVIGEHGDSEVLTWSIVDIGGLQLDDFVAAQKLTFTDADKEQIDEQVRRAAYVIIEGKGATYYGIGAAVANIVDVVAHGQKAILTICKPLKEVEGIADVTLSMPHLIHGKKRMMPLPLKLSQEERKALKQSASIIKKFLDDFKNGAS

SEQ ID NO: 63 - protein, 287 aa, Candidatus Abawacabacteria bacterium
MANVCKTEKIAIIGAGRVGTTFAFAALIRNIVAEVMLVDIDQERCKGEVLDLAHGLSHVNSGKVYQGTLKQAATADIIVITAGVAQKPGQTRLQLVETNAKIIKGILKEMGKINPMAILIIVSNPVDVLTYVAQKCSNLPAGQIFGSGTDLDTARLQYLLGKHFNMHPRSVNAFIIGEHGDSELAVWSSANVAGIPIKKTRGYSPAKMRAYMTETRSAAGKIIKLKGATFFAISMALIEICTAILKDQNLVLPVSTYIENYCGIKDVCLAVPAVIGRSGIKKLIKLP

SEQ ID NO: 64 - protein, 313 aa, Candidatus Abyssubacteria bacterium
MKQAKIVIVGAGAVGSTFAFTMMRSGLVGEIVLLDANRDRAEGEAMDLNHGLFFVPHVEVRVGEYSDCSGASIVVITAGAKQRPGETRLDLVQRNTTICKEIMRQVMEYTRDSIILMVTNPVDILTQVAYRISGLPSGKVIGSGTVLDSARLRFMLSRHCNVDSRNVHAYILGEHGDSEVAAWSLTHIGGIPILHYCSICKIDCGSEQRKRIADAVRDSAYHVIESKGATNFAVSLALENIVAAIVRDSNSVLTVSVPLKGEFGVSDVAMSVPVIVNREGVHHVLEPPLAEDELRALQRSASVLQDILRQITI

SEQ ID NO: 65 - protein, 310 aa, Candidatus Aenigmarchaeota archaeon
MRRKVSIIGAGFVGSTAAYSLLISGACSEIVLIDVNKQKAKGEAMDLKHGMQFVHQSKIRFGEDYRLCKGSSIVIICAGAGQKPGETRLDLVKKNAAIFKDMIPKITKHCKDCILLVVSNPVDVLTYIAMEYSGFPPERVFGTGTVLDTARLRYHLGEHYNVSASSVHAYILGEHGDSEFPVWSSARIGGAPLKSMKEYSKNDMDRIAKETKNAAYEIITTKGATYYAIGLVITKIVKAVFSDSNEVMPVSTRLDGYYGIRDVCLSVPCVVGSNGIDKQLLIPLNATEKRSLRKSANILRSTIKEVMVKK

SEQ ID NO: 66 - protein, 308 aa, Candidatus Altiarchaeales archaeon
MRVGIVGAGNVGSTIAYTLSMGSSVSEIVLADKNVDKAHGEVLDLRHGLPFIPYTKLEYGGLESLSNLDVVVLTAGIPRTHGESRLDLAGKNVGLFKEIIPQLAGQNKNAILLVVSNPVDIMTYVALKYSGFPKNRVFGSGNVLDSARFRSMLGHHFKVDPANVHSYILGEHGDSAFPFFSQAFIGCNPLKNMEGYDEREVREIFDRVKAVAAQVIKLKGATYYAVSLGVNKIIESIDLDKKRVMPVSTLIDRFYSGSELCLSVPAVVGKNGIEKILHVPFNEEEKTLFQASVEKIAKTIEEVGLSGG

SEQ ID NO: 67 - protein, 310 aa, Candidatus Amesbacteria bacterium
MKSTFKVSIVGVGKVGATAAYAMCLNGRATDLVLVAHQQETAEAEKLDLEHALPFLQHINIVATDSYEAVSGSDLIVITAGVAQKPGQTRLDLLQQNLQLFTEIIPKIYAASPESIVLIITNPVDILTYHSSQLAPFKPGQLFGSGTLLDTARFRFHLSEIFNVNPRSIHAYVLGEHGDHSFPALSAAHISGQPLSQFPNYSLEKVQDAFTQTQQAAYKIITAKGATYYAIATAILKLTNTIYSDAKSILPVSVPITNLYGVSGMALSMPCVVGQAGAEQVISIPLSNEEQAQFIQAADALKEAYRNVKK

SEQ ID NO: 68 - protein, 318 aa, Candidatus Aureabacteria bacterium
MKTVDVVINKVVIIGTGFVGSSIAFALMMSGRASEIVLIDANRKKAEGEMMDLNHGSAFTPPVDIYVGDYKDCKNADIIVIAAGANQKPGETRIDLVHKNTAIFKEIIPQITAVEKNAIMLVVTNPVDILTYVTLKVSRLLPEQVIGSGTVLDTARFRYLLSEHCGVDPRHVHAYIIGEHGDTEVPVWSRVIIGVTPLEHFCKLCHKKCNEEVKNAIFHDVKNAAYQIIERKGATYYAVALGVLRIIESILRNESSLLTISSYLDNYYGINDVCLSVPSLLRSEGIQKHIELPLNDEEHAALQRSADEMKNIIAQLDI

SEQ ID NO: 69 - protein, 307 aa, Candidatus Buchananbacteria bacterium
MSTKNKVTIIGAGMVGSTAAYSLIGDDSTQEIAMVDVNRKLVASQVMDLQHSVPFGSFTKVKVGSYSDIKDSKVVVITAGAAQKPGETRLDLVKKNSAIIGEIAPHIFKQNPKAIVVVVSNPVDVLTYQIIKMFPAKKNQIIGSGTVLDSARFRFLIGQKLDVNPRSVHAYIVGEHGDSELPLWSTAMIGNTFLDKFHKLSDREKKQIFDAAKNAAYAIIAGKQATYYAIASGITSIVRAILFDQKTVLPISHLLEGEYGIRNICLSMPAIVGAAGVIKKVNPEISAQEKKQLQKSAAQLKTVTKGL

SEQ ID NO: 70 - protein, 306 aa, Candidatus Cerribacteria bacterium
MRCDTRKVSIIGLGNVGATAAYALLLEGVVDELVLYSRTKEKAIGEKLDLEHGLNFLQPAKITATDSFDDVANSDVIVITAGVAQKPGETRLDLVKKNTEIIEALIPPLTKAAPEAIYVIVSNPVDLLTYKANILASLPKGRVFGSGTMLDTARFRYHLSEMLSINPRSIHAYILGEHGDSSFPVLSSASVGGQPLTTFPSYSQDQALQAFESARTAAYNIIQAKGATYYAIGVVIVKLVRTILQNSHSVLPISIPVEDYYGQYNVSLSVPCIVGRNGVEQILKAQLNEKEQEQFAKSATLLKSFL

SEQ ID NO: 71 - protein, 310 aa, Candidatus Collierbacteria bacterium
MLKSETFKVAIVGLGRVGMTTAYALLLKGLCTELVLFSRELAKAEGEKDDLTHGAPFYPHATVTATDKFEDLNGTDLVIFTAGCAQQPGQTRLDLTKQNCEIVAKLIPKIVREAPQTLILMVANPLDLMTLRATELAHLAPGRVFGSGTLLDTARFRLHLSKAISLNPQSIHAYVLGEHGDSSFATVTTATIGGKPLLSFPEMSPDHIAWSLAETRKDAGKIISSKGATYYGIATAVSHIVETIMRNSRKVLPLSTVLTGQYGLTNIALSLPCILGRSGVERVVDLPLSLEETASLHASAQILKTHLDEL

SEQ ID NO: 72 - protein, 317 aa, Candidatus Falkowbacteria bacterium
MFFKKSPKPVESTRVVIIGAGLVGATSAYAIMLQGIASEIVLIDIDKNKCAGEVLDLQHGISFLSPAKVWAGSYADCRDADVIVITAGLKQKEGQARLELAAANSKIVAEIMHKIIKYTSEAIILMVTNPLDVLTYVAYRASGFPANQVFGTGTALDSSRFRYLLAQSLGVAAESVGAYLIGEHGDSSVPVYSHANIMGGKLAVFPKYNKQAVQAAYRQTKNAAYDLICKKGATYYAIALAVARIVRAILYNENHIFPASVYLSGQYGISDVYLSLPAVVNRRGVKEILNIELSALEKKQLHQSAKVIRAAIDSIKI

SEQ ID NO: 73 - protein, 319 aa, Candidatus Firestonebacteria bacterium
MTKNLLKPKISIIGAGNVGMRYAYALAISGLARQINILDINKEKAEGEVLDLSHGAPYYSPVEIVYGEYDSLANSDLIVITTGKNQKPEQTRLELVKENVALYKNIIPAIMKYSPSSIILVVTNPVDVLAYTAFKLSGKPSKEVISSGTVLDSARLRFLLSKHFEIDAHNVHAYILGEHGDSEFPAYSSATVGGIHIKDYCLKCGDKSCNYQDELARIFKEVKSSAYGIIKRKGETSYGIGLALVRITSAIIKDENSVLPVSNLINGYLGIKDVYLSIPAIVNKGGVREVLDIKLDSKEEGQLINSANVLKNIIKDSGM

SEQ ID NO: 74 - protein, 301 aa, Candidatus Gracilibacteria bacterium
MSKKIVLIGTGMIGMSFIYSALQSDLASEYILIDIFTEYAEGNKLDVEDILPYNTKNISIKVGDYSDCSDANIIVICAGRPQKQGETRLEMIQDNAKIIKSIGVKVKDSGFSGISIIASNPVDILTFIYQQEYNFPKEKVIGSGCILDSNRLKVEIAKELNIFPHEVEAYVLGEHGDSSVMQFSNIKINGKKYDDFSEEKKVEIGNKVRNKAYKIIEAKKATYFGIGVALKKLCEDIIFDKKEIVSVGHFFEKDNKKLYISSPCIIGKKGIEEILNLDLSKKEQEEFKNSVGKIYKALKEY

SEQ ID NO: 75 - protein, 322 aa, Heimdallarchaeota archaeon
MRKLSPKVAIIGGGNVGIRYAYALMIKGLARHIIVVDIDIQKVQGEIMDLSHGIPYTSPVKLEVGAYEDIQGSDLVVITAGKNRKPGESRLELTKANVALYKEIIPQIMKYAPSALFLVVTNPVDILSYTAYKISNKPESEVIGAGTVLDTARFRNLIAAHCKVDPRNVHGYILGEHGETEFPVWSRVLVGGNLIKDYCPICENCDICNHEEELDKIFIEVRDSGAKIIKKKRETSYGIGLALVRITEAIFNDENAILPVSCLVNGFLDIHDVYLSLPAIITKNGVKKVLEIKLNEQEQLLLIKSANKLKEKIKEIMALLEK

SEQ ID NO: 76 - protein, 328 aa, Candidatus Hydrogenedentes bacterium
MDFSELNPKRKVVVIGAGSVGATFCYALAQSGLADEIVLIDHNKDLARGQVLDLAHGQSFFPPVTIRVGDQQDYADATLLVMTAGARQQPGETRLQLLRRNASIVRQVARDIALANSPGTLVIVSNPVDILTKVAAEETGWRRGRVLGSGTVLDSARFRSLLSHNCGIDIHNIHAYILGEHGDSEFAAWSMTHVAGIPIDEYCTSCRMCTPTGKQDEWLGVRKSIEEQVRNSAYHIIDYKGSTYFAIGLALVRIAGAILRNENSVLTVSTLLEGEYGVSGLCLSVPAVVSGRGVERIMEARLNPEEQKALARSAAVLRASLNELEGNE

SEQ ID NO: 77 - protein, 306 aa, Candidatus Jacksonbacteria bacterium
MNNKITIIGAGMVGSTTAYSLLASNNVGEIALIDINQKLAHAQAMDLQHSVPFLGYTSIHNGTYADIKNSSIVIITCGAAQKPGETRLDLVKKNSAIIKDILIKVYHQNPHVIIIMVTNPVDILTHIACTLYPKNKSCIIGTGTILDSARFRFLLGEYLHINPQSVHAYIVGEHGDSEVPLWSTATVGNTPIEKVKKLSATVKKEIFENAKNAAYAIIEGKQATYYAIATGVAMLVDVITHDKKTVLPVSRYINGEYGIRNVCLSMPAVIGKEGIISTIPLTLSSQEKSALKKSAKTLQSILKATD

SEQ ID NO: 78 - protein, 306 aa, Candidatus Kerfeldbacteria bacterium
MSNNGKVVVIGAGFVGATSAYAMFIDGAPSEIVLLDVNKEKAEGEAMDLEQGMQFVPGTKLSYGSDYALVRNAEVVVITAGARTKPGQTRLELISVNAQILKTIIQNIKKYNKDCCLLIVTNPVDVLTYLAVRYSGFSYDKVFGSGTTLDSARLRYFLGQKLRVHPSSIHAYMLGEHGDSEFPAWSSARVGGVPVLEMEGLDRAILNRLADNTRRAAYEIVARKGATYYAIGLVVAQLVRAILDDSNTIFPLSVYLKKYHGVSDVTLSVPVVLNRSGAHIRFQLPLSQQEKKQFRSCAKIVRSLQS

SEQ ID NO: 79 - protein, 308 aa, Candidatus Komeilibacteria bacterium
MLLKNKVTIIGAGMVGSTAAYSLIASNLLEELALIDSHPAYLKAQVMDLQHAIPFHGNTQVKAGTYEDVRDSRVVVITCGAKQKVGETRLDLVKKNSAIIKEILPRVFKANPRAVVIMVTNPVDVLTYLAVSLYPKCARQIMGSGTILDSARFRFLLSQKLQVSPKSIHAYIVGEHGDSELPLWSNATIGGGGIEKFAGLSAAAKKSLFNQAKNAAYAIIAGKQSTYFAIASGVAEIVGAVIMNRRTVLPVSHLLTGEFGLKKVCLSLPVVVGREGIAQKVGLTISPAEKKQLVESARKLKQVFRSVK

SEQ ID NO: 80 - protein, 321 aa, Candidatus Latescibacteria bacterium
MQDTSGSRRKVVVVGAGAVGATFAYALAQSGLADEIVLIDRNEDLVRGQVLDLAHGQPFFPTVSIRIGDASDYSSASLIVITAGAAQRPGETRLQLLQKNAAVIKGVMTDIVEQASPAVVLVVTNPVDVMTYVALETSGWDRSRVIGSGTVLDSARLEHLLSAHCGVDVHNVHGFVLGEHGDTEFVAWSLTHIAGMQMDVYCPICKGCADNLAEREAITQQVRDSAYHIIGYKGATWFAVGLALVRIAGAILRNQRSVLTVSALLHGEFGLSDVCIGVPCIVSARGIERVVESALSESELAALHSSARTLRKAVEQLHAGA

SEQ ID NO: 81 - protein, 304 aa, Candidatus Levybacteria bacterium
MGSKVTIIGGGHVGTSAAFAMLLRETAREIVLLDRDKNKMMGEQLDFQHSLAFLATTKIVAAQSYEDTKDSDVIIFTSGVAQVSGQSRLDLLKSNAEILEATLPGVVKLSPESVVIIVSNPVDALTYKASRLLNLPKGRVFGTGTSLDSARFRFYLSELLSINPKNIHAYVLGEHGDSSFPVISTADVGGQSLINMKGISKEQIQECFIKTRDAAKTIIATKGATYYAIGVVISQLTHAVLEDAKRIFPVSIPLDGEYGQKGVSLSVPCELGRKGMEKILEIPLSDEEKRLMENSANILKKFIN

SEQ ID NO: 82 - protein, 316 aa, Candidatus Liptonbacteria bacterium
MASKPNKTPIESTRVVIIGSGLVGATSAYALMLQGSASEIVLVDIDKKRCAGEVLDLQHGSSFLPEVKIWAGDFSDCKEADVVVITAGLKQKENQSRLELAKTNAKIVSDITKNITKYTKKAVILVVTNPLDIMTYTAWRASKLPKNQVFGTGTVLDSSRFRHLLAEKIKIDPESMGAFLLGEHGDSSVPVFSHANVMGEPISSLKKYGKINTEDAYKKVRNAAYELISKKGATYYAIGLVVARLVRAILYDENHVFPVSVYADGHYDLKDIYLSLPAVVGRNGIKQIIEIKLSDQEKNLLQKSAAIIKQALKELE

SEQ ID NO: 83 - protein, 306 aa, Lokiarchaeum sp.
GNVGMRYAYALMIKGIARKIVLVDLDKERLYGEVMDLSHSTPFTSPVEVISGDYSDIRDSELVVITAGRKQKPGQSRLDMAKGNVSLYENMIPEVRKHAPSAIYLIVSNPVDILTYAAYKFSKKPASEVIGSGTVLDSSRFKYLLGKHCNVDPRNVHAYILGEHGDTEVPIWSKAMLGGGALIDYCPTCKNTMTCDREEELNTIFEEVRDSAYEIIERKGETSYGIGLSLVRITQAILNDENSILPVSCFIDDYIGIQDVYLSLPAVVNKEGIRDVLKLELDKGEQEKLRFSAYTLKNVLKEVGLN

SEQ ID NO: 84 - protein, 309 aa, Candidatus Magasanikbacteria bacterium
MDNKKPLATKIAIIGAGSVGSTIAYVATLKNLAAEISLIDINVKKEEGEVMDIADGMCFVETGCVKGTDFASARDADIIVYTAGAPQAPGETRLDLATKNRNILKSVFKKIARFKNTAIVIIVANPVDALTAEAIRLTQLPRGRVFGTGTALDTARLRTELSHLFKISAQNVHGFVLGEHGNSEFVAWSSVTIGGIPTAKLKLLTAHARTEIETRVRQEAYEIISRKNATFYGIGLITADIIEAVLFDQKKILPISILVENWNDVDNIVLGVPAILGRAGVEKIWPLILSKQEQKKLTASAAMLKKYEV

SEQ ID NO: 85 - protein, 280 aa, Candidatus Gastranaerophilales bacterium
MNDIKETVNFNKAVIVGCGFVGSASAFSLMQSGLFTELVLIDSDSKRAEGEALDISHGIPFSKPMKIHAGDYDDVKNAGIVIITAGANQQPGETRLDLVKKNINIFKTIIPEIKKRNFNGILLIVANPVDILTYAAVKLSGLSENRVIGSGTVLDTARLKYAIGRHLNVDSRSVHAFIIGEHGDSEIAVWSSANVSGVPLNNFCEMRGHYDHQNATEKIATDVKNSAYEIISMKKATNYGIAMSVKRICEAIVRNERSILPVSTIMHGEYGISDVSLSMP

SEQ ID NO: 86 - protein, 307 aa, Candidatus Microgenomates bacterium
MFKQETFKVAIIGLGRVGITTAYAILLKGLATELVLFSREIEKAEGEKADLEHGMPFYPKCNIIASSNYEDLSGTDLVIFTAGCAQKPGETRLDLAKNNCAIVDALIPNIVKHAPHTLILMVANPVDIMTLRAVEKAKLPEGRVFGSGTLLDTARFRLHLSKGVKISAKSIHTYILGEHGDSSFAATSTATIGGKPILSFPEMSPEHIQWAQDQTRKDAYKIINGKGATYYGIASAVTHIVETIMRDSKKIIPLSTPLTGQYGLDNVSLSLPCILGRNGVERIIDLPLSVTETAALHNSAKMIRQSI

SEQ ID NO: 87 - protein, 309 aa, Candidatus Moranbacteria bacterium
MLMKNKVTIIGAGMVGSTVAYSLILQDIVDEIALIDLNEDLVKSQVMDLEHSIPFVGRTDVKVGDYDDCADSAVAVITCGAAQKPGETRLDLVQKNAAIIKKVIPAIFDKNPDIILVMVTNPVDVLTHVAVSLFPEKKDQIMGTGTILDSARFRHLIGKKLDVDPKSIHAYILGEHGDSEFPVWSTASIGNMQIGTCDCISPEEQENIFTQARGAAYTIIEGKQSTYYAIGAGCAHLIRAIVRNKKSVLPVSHLIEGTYDINDVCLSMPAIVGYTGLMGKLCIKLNKTEQKQLKKTAEVLKETFAKIEN

SEQ ID NO: 88 - protein, 310 aa, Candidatus Nomurabacteria bacterium
MANKSSKVVIIGAGFVGSTAAYALLIDGTASEIALIDVDREKAEGEALDLKHSLQFTSQTKITFGEDYNLCKDAAIIVICAGAHQKPGETRLDLAQKNAKIFKEMIPKITRHNRDCILLIVANPLDILTYLAIKYSGFPSHRVFGSGTILDTARFRYLLGEYFEVDTTSVHAYILGEHGDSEFPVWSTANIAGINLRLFDNYNKKKMGEIFKKTRNAAYEIIAKKGATYYAIGLGITKIVKAILKNHNEVLPVSCLLKNYHGISDVCLSVPAIINKDGIKKQLKLPLNPQEKANLRKSANVLKNIIKKVV

SEQ ID NO: 89 - protein, 318 aa, Candidatus Omnitrophica bacterium
MENLRPKVSIIGCGNVGMRYAYALIIRGLVRQIVIVDIDRQRLEGEVMDLSHGAPYISPVEIIAGDYPDIKNSDLVVITIGRKQKPGQSRTDLARDNVELYRKVIPEIVRYAPKSIILVVTNPVDVLAYAAYKISGKPAKEVISSGTVLDSSRFRFLLSKHCNIDARNVHAYILGEHGDSEFAVWSKAMIGGILFKDYCRICKTNNTCSSKEELNKIFLEVRDSAYKIIEKKGETSYGIGLTLVMITEAIINDENAILPVSSLVDGYLGIIDVYLSLPAILNREGVREVLEIELSPQEEKALINSANSIKKVIKEVGL

SEQ ID NO: 90 - protein, 319 aa, Candidatus Pacebacteria bacterium
MENKNYKVNCKAREDALGYKISIIGCGKVGMTTAYSILHDGVVNDLLLVDRNKSKIIGEQLDLEHGLSFLHHAHIDATDDYANIKGSDLVIITAGVAQRPGDTRLDLANKNLKIIGEVIPKIVQHSPESIILIVSNPVDVLTYKAYQLAGLPKGRIFGSGTTLDTARFRFHLSEFLKVNPRSIHAYILGEHGDNSFPVISSASVGGQPLATIPGFSEERAEKAYSKARDAAYKIIASKGATYYAIGAVVAHISRMVLTDDKSILPVSIPLHGYKDISGIALSVPCIVGRDGVEKILDVKMSWDEKKKLQNAAEVLKKLL

SEQ ID NO: 91 - protein, 315 aa, Candidatus Peregrinibacteria bacterium
MLPCGHTAKIGIIGAGFVGTTFAFAAMIKNLAARIVLVDANQEKCEGEVMDLAHGLNFVETSQIMHGNYQDLADADAVVVCAGRGQRPGETRLDLLQDNVKILKSILEEFKQLHNQTCILVIVANPMDALTYVAKKLSGLPENQVFGSGTVLDSSRLRFLLGEYFEVSSQSMKAYVFGEHGDSEFPVWSHANIGGKPLQDFARYDAQKMEEIFQQTKNAAYEIIKRKNATYYGIALALTDIVESILYDQNKVLPVSHTLADYYGTKDVCLSLPCVVCRRGIKETLDIPLNEEEVQKLHSSATTLRQSLDSIQNLL

SEQ ID NO: 92 - protein, 308 aa, Candidatus Roizmanbacteria bacterium
MKSNKVVIIGGGRVGMSAAFAMLLKEKVGEIVLYDRDIEKMKGEQLEFEHSLSFLGSTKITVASSNNDFENSDVIVFTAGVAQKPGESRLELVQKNTEIVKDILPAAVSQSPNAVLIMVTNPVDVLTYEASKILNLPKGRIFGTGTSLDTSRFRFHLSEILKINTKNIHAYILGEHGDSSFPVVSNADVGGQQLLSVPGINEKIINDCYIKVKEAAQAIIQSKGATYYAIAVVVSELVEAVLSDSKRVYPVSVPLDGQYGLKDVALSVPCVIGRNGVEEILEIDLSSIEKQNLDKSSEILKEFNGKKT

SEQ ID NO: 93 - protein, 308 aa, Candidatus Saccharibacteria bacterium
MNKQKLVIVGAGGMVGATAAYACALRSVVEEIVLIDRDPDLAWGQAADITDGMGIDRCVVVRPGSYDDIKTDDIVVITAGAPQQPGQTRLELLGVNAEIMRGTVRNIMRNGARPYILVVSNPVDALTYVALKESGLPKSRVFGTGTTLDTSRLKSYIADQLDVHSREVDAYILGEHGDSSFATIESAQVGEVPLADYPGFKPAMVDGIEEQIRQRAYRVIETKRSTYYAIGFVISKIVSALRSSSRSVYPVCSLVEGEYGLHDVVLGLPSTICADGVKILTGYPLNEREQAALRHSAKVVTEAIRSLE

SEQ ID NO: 94 - protein, 322 aa, Candidate division BRC1 bacterium
MERHSWAKRRKVAVVGAGAVGSTFCYALAQSGLAEEIAVIDRNENLVRGQVLDLVHGQPYFPTVSIRVGDASDYADAQLIVITAGAAQRPGETRLQLLQKNAAIVRGIVDDIFARESAATIVIVSNPVDVLTAVAQKRAGGARGRIIGSGTVLDSARFRYLLSQRCGVDIHNVHAYILGEHGDSEFAAWSMTHVAGMPVDEYAQLFRPSEDWAAERRQIEREVRDSAYHIIEYKGATCFAIGMALVRIAGAILRAQRSVLTVSVALEGEFGLDDVCLSVPAVVSEGGMAKIVESALPDNEREALFASAAVLKQAMSQLDRDE

SEQ ID NO: 95 - protein, 314 aa, Candidatus Woesearchaeota archaeon
MEATMAKRTGKVAIIGAGFVGSTAAYALLIEGAASEITLIDRHLQKAEGEAMDLRHGLQFRADSRVTYGTSYSLCRDAEIIVVCAGAHQEKGETRLDLVKKNAAMFREMIPSIVKHNKDCILVVVSNPVDILARLALTYSGFPASRVFGTGTMLDTARFRFLLGERFGVSPESVHAYILGEHGDSSFPVWSTANIAGVPLRDFRQYDKRAMEGIYQQTKNAAYEVIARKGATYYAIGLAVARLVKAILSDQNMVFALSALLKGYHGVNGICLSVPCVVNREGIREQIVMPLNAEEKKKLKKSAGVMKGILRGIN

SEQ ID NO: 96 - protein, 305 aa, Candidatus Yanofskybacteria bacterium
MENTMSKIAVIGAGSVGATTAYTLVMKNLAAEVILVDINEAKEEGEVMDINDALSFVETGKIKGGSYEDAAMADVIIITAGLPQKTGEQNRLELVNKNKEIIRSIFGQLKPLNPSAVIVIVSNPVDIMAYYAQELSGLPRTQVFGTGTSLDTARLRTEIGLALDVNPQSVSGFVLGEHGESEFVAWSTVNVGGVPIREKLSQDRIDEIAQKVKDDAKNIIDRKGATFYGIAAVVSDVVESILLDQDKVLPISTRLENHSGISGVCLGMPAVIGRQGIKEIWNLELVGSEKEKLRQSAEAIRQYIL

SEQ ID NO: 97 - protein, 312 aa, Candidatus Anoxychlamydiales bacterium
MQPKQKKISIIGAGSVGSSYAFSLMMSGIAREVVIVDINKKKAFGEALDLSHVQSFISPVEISYGNYEDIKDSDIVVITAGLNQKVNQSRLDLVKDNTKIFKEIIPKIAKNAPNSILIVVTNPVDVLSYVAYKISDFPKEKVIGSGTVLDSSRLRSLLSNFYKIDARNIHANLIGEHGNTEFPVWSKANISGIPFDKCNLIKYKKEDLEKIFEEVKNSAAKIIEAKGSTCYGIAISLLKITKSILRDENSILPVSSFIDNYLDVNDVYLSVPALIGSQGVKGILKMDLSNDEINNFHLTAKTIKDVIKQIGF

SEQ ID NO: 98 - protein, 305 aa, Chloroherpeton thalassium
MKVGIIGAGFVGATAAFAMAMRGSCSEIVIVDADNAKAKAQASDIEHAVPFSFAMTVRDGDFQDLKGAKVIIISAGVNQKPGETRLQLLERNANIFRDIVPKVVAIESNAVIVVATNPVDILTSLTEQLAGLPEGQVMGSGTTLDTARFRALIGNELGVDPQHVHAYVIGEHGDSEVFAWSSANVAGLSIPSFCKARQVRWNEEIQSQIADNVRKAAYHIIEGKGATYYGIGAVLARISEALIRNHRAVLTVSANIPEFGVALSLPRLVSGKGIDGLIGVQTNDEERAALERSASVLREALSAIS

SEQ ID NO: 99 - protein, 319 aa, Bellilinea caldifistulae
MTHVFKKPTRVAIVGAGNVGATFAYSLLISGLASEIVLIDANHAKAEGEAMDLNHAMPLGRPARIWAGSYEDTAGAVITVITAGSAQRPGETRLDLVQRNTEIFKQIIPKIVENNPNGILLIATNPVDILTYVAFKISGFRRNHVIGSGTVLDTARFRYLLSQHFDVDPRSVHAHIIGEHGDSEVPVWSLANIAGMRLPQYCAVNELGCADETLNTIFEQTRDAAYHIIERKGATYYGIASGLVRICEAIIRDQGTVLSVSSYIDEPYYGIEDVCLSLPTIVDLDGVERIIRLDLNEEEVIGLQKSANLLKNIISQLKI

SEQ ID NO: 100 - protein, 291 aa, Mantoniella antarctica
MATPACSSGVRAIGYAGATHRGSRDSAYPRACVPASVRHVNREETLQLLSRSRRCKSACVVQATGSVSLREDLFGSKEPLFTDCRSSKVSIVGSGQVGLACAYALINQATCRQIVLHDIAPKMDRLEAEVADLLHGAEFVDSLDVVATADFADTADSDIVIIPAGARQNEGESRLALVARNVAIFEDIIPKIAAASPDAKLLILTNPCDIMTHVALRLSGFPSNRVIGSGTALDTSRFRSLLAHKLAVDTGSVHGMVLGEHGDSSVVLWSQVMVGGGDFEPAYSYILYPEP

SEQ ID NO: 101 - protein, 332 aa, Homo sapiens
MATLKDQLIYNLLKEEQTPQNKITVVGVGAVGMACAISILMKDLADELALVDVIEDKLKGEMMDLQHGSLFLRTPKIVSGKDYNVTANSKLVIITAGARQQEGESRLNLVQRNVNIFKFIIPNVVKYSPNCKLLIVSNPVDILTYVAWKISGFPKNRVIGSGCNLDSARFRYLMGERLGVHPLSCHGWVLGEHGDSSVPVWSGMNVAGVSLKTLHPDLGTDKDKEQWKEVHKQVVESAYEVIKLKGYTSWAIGLSVADLAESIMKNLRRVHPVSTMIKGLYGIKDDVFLSVPCILGQNGISDLVKVTLTSEEEARLKKSADTLWGIQKELQF

SEQ ID NO: 102 - protein, 307 aa, Spizellomyces sp. 'palustris'
MPAKIAIIGGAGSVGATAAYAILLRRCASELLLVDLDTEKCAAQVLDLSDAAFLSDTKVRMGTPKEAGQCDIVIVTAGAKQRPGETRVDLIGRNRAILSSVIESMKPFKQSTILLLIANPVDVLTYFAQKLSGLPQSQVLGSGTYLDSARLRSELSSRLEVAETAVHAYVLGEHGDSQFVAWSSAHVANTPLLSLPAMKGVDRKKLAEDVKNKAYKIIEAKGATYFGIGGVAASICECIIFDLRHIRPLSHFIPELNVCLSFPVVLGHSGVKQTLKPPLTDEEEELLKKSAKEMRTIIEKYELAPNP

SEQ ID NO: 103 - protein, 332 aa, Stylophora pistillata
MATVQEKLMTKVYEEERAAPSKVTVVGVGQVGMACAYSIMQQGICRELALIDMIEDKLKGEMLDLQHCQRFVKNVSIHASTDYAVSANSNLCIVTAGSRQKEGESRRDLVQRNVNIFKAIIPQLVKHSPNTILMIVSNPVDILTYVAWKISGLPHERVIGSGTNLDTARFHFLISEKLNIAPNNVHGWIIGEHGDASVPVWSGVNIAGVNLKDLHPDIGSDGDLEKWNEVHKKVVNSAYEVIKLKGYTSWAIGLSVSTMTQALLRNQKNVHAISTLAKGFHGIEDDVFLSLPCVLGSHGVMYVIKQTLDENETKQLQTCARTMNELQQSLQF

SEQ ID NO: 104 - protein, 310 aa, Crenarchaeota archaeon
MKISIIGSGRLGSTTAFELINRELASEIVLVDIIPNLPQGEAMDLNQMSAEKGKNIVVYGSNDYKDIKDTSIVIVTAGVARKPGMTRMDLLKTNAPIVRDVTKEIVKYAKDSIIIVVTNPMDVMTYVALKTSNFERNRVIGMGGQLDSARYREILSQMLNISRSSIKALVIGEHGETMFPIPRFSIAGYKRVSELLDAEKIKEAEEKTRKIAAEVIALKGATVFAPISCIATLVESIVKDKKDMLPVSAYLQGEYGVKDVCIGVPAIIGRNGIEKIIELDLNEEEKARFGASVNTIRKAIEEILTLKIIE

SEQ ID NO: 105 - protein, 331 aa, Microcystis aeruginosa
MLDKIFTPNPYAEQPAPLRPRKGVIIGVGQVGMACAYSMLIQDCFDELILQDIATDKVEGEVMDLRHGMPFIEPTDLKMGTVADVGQNADVVIITAGAAQKEGETRLHLLERNVAIFRRILEDVAVYCPSALILVVSNPVDIMTYVTLKITNFPPSRVIGSGTVLDSGRLRSLLSTQLHVDARNVHAYIIGEHGDSELAVWSSANIGGARLLEGDWQDLSAANQESLTEIFLQVKNAAYEIIKRKGYTSYAIGLATTDIVKAILRSQERILTISTLLDGQYGLKDVCLSIPSVVNEKGVIKTLNLALSPRETQQLHNSAKIMRDLIDQLEI

SEQ ID NO: 106 - protein, 310 aa, Thermus caldophilus
MKVGIVGSGMVGSATAYALALLGVAREVVLVDLDRKLAQAHAEDILHATPFAHPVWVRAGSYGDLEGARAVVLAAGVAQRPGETRLQLLDRNAQVFAQVVPRVLEAAPEAVLLVATNPVDVMTQVAYRLSALPPGRVVGSGTILDTARFRALLAEHLRVAPQSVHAYVLGEHGDSEVLVWSSAQVGGVPLLEFAEARGRALSPEDRARIDEGVRRAAYRIIEGKGATYYGIGAGLARLVRAILTDEKGVYTVSAFTPEVEGVLEVSLSLPRILGAGGVEGTVYPSLSPEEREALRRSAEILKEAAFALGF

SEQ ID NO: 107 - protein, 318 aa, Dictyoglomus thermophilum
MKKILIVGAGAVGTSFAYSLIHKGLVEEIVLYDIDEKKAKGEALDLAHGIYFTKPVEVRAGGLEEAKDSDIVVITAGAKQRPGETRLQLLDRNISIYKDLVPEIVKNGFKGIFLIVTNPVDVLTYFAYTFSGFPRNRVIGSGTVLDSSRFAYLLSKHCDVDPRSVNAYVIGEHGDTAVLAWSLTHIGGISISEFCPVCGRRCFDEDVKKAIIKEVRDSAYKIIEYKGATYYAIGLALVNIVEAIVRDENRILPVSTVHPQIFEFKDVPLSLPSIVGRNGVKKVLRVKLTEEEEKELYNSAKFIKEAIDSFSSLSLSSR

SEQ ID NO: 108 - protein, 371 aa, Strongylocentrotus purpuratus
MTTITSKLMDMVVDHLDDSSPTKVTIVGVGQVGMACAYSIMTQNIASEIALVDVIADKLKGEVYDMQHGQAFVKGCSVKGDTDYKVTAGSRLCIITAGARQREGESRLNLVQRNVKIFEGIVPNLVRYSPNTVLLVVSNPVDILTYVAWKLSGLPSNRVIGSGTNLDTARFRFLLGEKLGIAPSSVHGYIIGEHGDSSVAVWSSTTVAGVSLQQLDPEIGTVKDPENMHQVHQEVIDSAYEIIKLKGYTSWAIGLSCATLAAAVLRNQKGVYAVSTVAKGYHGIEHPVFLSLPCILGQDGITHVIKQTLNTKEQAQLQASANTLWDIATSLDIREPSKYTNMLMGIGHFVMWTFVPLVALFAGHRAGHGRG

SEQ ID NO: 109 - protein, 320 aa, Endomicrobium proavitum
MADKLSPKVSIIGCGNVGMRYAYSMIIKGAARELVLVDYNRQKAEGEAMDLSHGAPFVSPINIYAGDYPDTANSDLVVITAGRGQKPGETRIDLIKGNAEILKSVVPQVVKYSPKAIILVASNPVDILSYITYKISGKPANEVIGSGTVLDSARFRFLIGKHCNVDSRSIHASIFGEHGDTEFPMWSKAMIGGVLFKDYCKVCNKENCAKQEDAKLNEIFEDVRDSAYEIIAKKGETSYGIGLALTKISKAILKDENSVLPVSSLLDNYHGVSGIYLSVPAVVNKGGIRQTLQVDFDMVELDSFINSAEQVKKVIKASGF

SEQ ID NO: 110 - protein, 316 aa, Methanophagales archaeon
MPVSRSKVAIIGTGNVGSTFAFALMISGLAREIVLIGRDKKRAEGECMDLNHGASFVPPVTIYAAGYEGCAGADVVVITAGARQQPGESRLDLAQRNADIFKDIIPRIAEHAENAILLVVSNPMDVLTYLTIKLSGFSPQSVIGSGTVLDSSRFRFLISQQCQVDPRNVHAYIIGEHGDTELPVLSHANIGGMLFPQYCARCNRRCDYKEEFGRIFEEVKNAAYQVIEAKGATYYGISVALIRIVAAILRDENSVLPISTLLHDYYGIEDVCLGIPAVVNRSGVERVLLLELSPTEQELLRHSARTLKEVIRGINL

SEQ ID NO: 111 - protein, 317 aa, Geobacillus stearothermophilus
MKNNGGARVVVIGAGFVGASYVFALMNQGIADEIVLIDANESKAIGDAMDFNHGKVFAPKPVDIWHGDYDDCRDADLVVICAGANQKPGETRLDLVDKNIAIFRSIVESVMASGFQGLFLVATNPVDILTYATWKFSGLPHERVIGSGTILDTARFRFLLGEYFSVAPQNVHAYIIGEHGDTELPVWSQAYIGVMPIRKLVESKGEEAQKDLERIFVNVRDAAYQIIEKKGATYYGIAMGLARVTRAILHNENAILTVSAYLDGLYGERDVYIGVPAVINRNGIREVIEIELNDDEKNRFHHSAATLKSVLARAFTR

SEQ ID NO: 112 - protein, 314 aa, Cetobacterium ceti
MKTRKVGIIGVGHVGSHCALAMILQGACDELTLVDIDKQKAKSQAIDCMDTISFLPHRTIIKDGEIDDLTDMDIIVISVGNLTADKNRLNELKGSIEMVKSFVPQIVKNGFKGIFVVITNPVDIVTYYVQKLSGFPHNRVIGTGTGLDSARLRKVLSQTTNVDPRSIQAFMLGEHGDSQVANFSTGTINCKPILDYLKENEDTIGKLDLDQLEHKVAQGAWDIYAGKNCTEYGIGCTCSDLVQNIFHNERRVIACSAYLQGEYDYEGIYIGVPAIIGKDGLETIIELPLDERERTKFKKSCEIMSSYIEMAKNY

SEQ ID NO: 113 - protein, 305 aa, Gemmatimonadetes bacterium
MTISVGVVGTGWVGSSVAISTLHGGFASELLLADVRHDLAEGEAMDLAHGAAFYTTASVRAVPIDEMLHTDALVVAAGRGGKPNESRLDLLRDNAKILRELGEKLRGYRGLVVVVTNPVDVLTYVVAESSGLPCERVIGTGTMLDTARLRQVLGHELRVDPHSVHAQVVGEHGDSEVVLWSSAHVGGTPLREWPGWSREREQPIATEVRTAAYEIIKRKGATNHAIGLTTAALLRSALRGERRVLTVSRVQSGVLGLRDVALSLPTVVDAGGAVDVIPVKLDDAERHGLDRSADVLRQAIASLRE

SEQ ID NO: 114 - protein, 314 aa, Ignavibacteriales bacterium
MKVGIIGSGMVGATSAYAIMLRKAASEIVLIDSNEKRAQAEAADIIHAAPFTQATVVYAGNYSDLKGAKIVVIAAGAHQSPGETRLMLMEKNASILNDIISKVAEVAPNAIFLIATNPVDIITYISISIAKNYGIPATRIIGSGTTLDTARFRSLLGSHIGVDPQNVHAYVIGEHGDSEVLTWSNIDIGGVPLEDLIEYRKIAFSEKIKEEIDKGVRNAAYKIIEGKGSTYYGIGGAIAKLVDVINRDNRSVLTISTYEEDVEGIKNVALSLPHLIGGEGDLGVLPIRLNMKEKLLLKKSAEVIRSKIDEYEVK

SEQ ID NO: 115 - protein, 321 aa, Lentisphaerae bacterium
MPQPSVHRRKVVVVGAGAVGSTFAYALAQSGLAEEIALIDMNTDLAKGQVLDLVHGQPFFPTVAIHVGTPADYADAHLIVLTAGAAQRPGETRLQLLQKNAAVVRAVVRDIAAQDSRAVLLVVSNPVDVMTAVALHETGWERHRIVGSGTVLDSARLRHLLSAHCGVDVHNVHAYVLGEHGDSEFVAWSMAHIGGLPMREFCPLCRHCEDWQAERRRIEQQVRDSAYHIIGYKGATWFAVGMALVRIAGAILRGQHSVLTVSSRLDGEFGLRDVCLSVPCVVASNGIERLIESTLPSDEQAALEASAAKLREAIGQVIGPA

SEQ ID NO: 116 - protein, 302 aa, Rhizopus microsporus
MVSHSKVAIVGAGAVGASTAYALMFKNICSEILIVDINPEIVQAQVLDLADAASVSHTPIRGASTEEAGQADIIVITAGAKQKEDEPRTQLIERNYRVLKNIIGSMQPIRPDAIILLVANPVDILTHIAQRLSGLEPNQVIGSGTYLDTTRLCVHLGEIFDVNPQSINAFVLGEHGDSQMIAWEAATIGGQPLTSFPEFQELDKQAISRAISGKAMEIIRLKGATFYGIGACAADLVHTIMLNKKSVHPVSVYVEKYGVTFSMPAKLGWKGVEKIYEIPLSEEEETLLLESVKALQEIERLY

SEQ ID NO: 117 - protein, 377 aa, Meloidogyne enterolobii
MAENGIFVPVAPIESTPQNKVTIVGVGQVGMACAYSILQQNIATEICLTDVLADKLQGEMMDLQHGLAFTHNTCIVNASTDYAKTAGSKICVITAGCRQREGESRLSLIERNVVIFKGIIPQLVRHSPNTVFLVVSNPVDILTYVTWKLSGLPKERVFGSGTNLDSARFRFLLSERLNISPCNCHAFIIGEHGDSSVAVWSGVNVAGVNLSAQDLTTGTSNSNAKNDDGKLEEEIHKKVVQSAYEIIRLKGYTSWAIGLSVASIVQGVMRNSRNVFALTVNIKGIHGFEDDIFLSLPTVLGSNGVNFIVRQNLTPKELEQLRGSATQLLEIQKNFEALNNMGNNDKYVVGNILNIQYFFPLNSVVSLNFFYFYLTIN

SEQ ID NO: 118 - protein, 312 aa, Nitrospirae bacterium
MGHTHRVAIIGCGRVGATTAFALLHTGQVEELVLIDTDRARAEGEAMDLAHATALLAPARVWAGDYADAASAAIVIVAAGRASASRDESRLQLVGDNVRITRQIVGELAAVGFSGCLLMATNPVDVLAQIAASASPLPAARVIGSGTLLDTARLRQLLATACALDPRSVHAHILGEHGDSEIVAWSSAAIAGMPWAAFGAQAGVELAPEAILDSVRGAAPAIIERKGATNFAIGAALARLVSCILRDEHSVLMVSTRLAGEYGERDVYLSVPCVVGGGGVERIIELDLSPAEWAGLHRSAEILRDVARRVAA

SEQ ID NO: 119 - protein, 333 aa, Trichomonas vaginalis
MSEAAHVLITGAAGQIGYILSHWIASGELYGDRQVYLHLLDIPPAMNRLTALTMELEDCAFPHLAGFVATTDPKAAFKDIDCAFLVASMPLKPGQVRADLISSNSVIFKNTGEYLSKWAKPSVKVLVIGNPDNTNCEIAMLHAKNLKPENFSSLSMLDQNRAYYEVASKLGVDVKDVHDIIVWGNHGESMVADLTQATFTKEGKTQKVVDVLDHDYVFDTFFKKIGHRAWDILEHRGFTSAASPTKAAIQHMKAWLFGTAPGEVLSMGIPVPEGNPYGIKPGVVFSFPCNVDKEGKIHVVEGFKVNDWLREKLDFTEKDLFHEKEIALNHLAQ

SEQ ID NO: 120 - protein, 303 aa, Stieleria varia
MKITIVGTGKVGSAIAFANVMNPMASELMLVNRTREKAEGDALDLSHASALRNSNMRISAGDIPDSEGSDIIVFTSSVPYGDPNRKRSELASDNHALLKEWIPALAKFSPGAVLIIVSNPVDALTYAAIELSGFDPCRVIGTGTLLDSVRYRAMLSDTLKIHSDDIRAYILGEHGDTQFAASSIAMTGGERFYPNDVSQQIFQRTVGMGYQVSKLKGYTNYGIALATMQILDSIVYDLRHTMPLSVLIDGFCEVTDVCLSLPAVIGREGVTRVIRPQLTAEEQDAFRRSAESVRKTISLMRAV

SEQ ID NO: 121 - protein, 380 aa, Pusillimonas sp.
MTCVEDFRRLAMRRVPRMFYDYADSGSWTESTYRANETDLERLKFRQRVAVNIESRNLRTSMIGEDVAMPVAIAPTGLTGMQHADGEILGAKAAEAFGIPFTLSTMSICSIEDVAAHTSRPFWFQLYVMRDRDFIGRLIDRARAAACSALVLTLDLQVMGQRHKDIKNGLSTPPKPTLANLLNLLTKPRWCIDMLGTQRRGFGNIIGHAKGVSDVGSLSAWTASQFDPTLSWNDIEWIKKRWGGKLILKGVMDAADARIAAQCGADALVVSNHGGRQLDGAPSSISALPAVVQAAGKDIEVFVDGGIRSGQDILRAVALGARGTMIGRAFLYSLGAMGQPGVQRCLQMLANELDVSMAFCGHTDIRKVDRSILVNGDIFD

SEQ ID NO: 122 - protein, 354 aa, Cyanidioschyzon merolae
MTSGIDEAAAELQGSLFGDVSPAIDTPGAALARSYPVRITVVGAGDVGVACAYNILTRDICSELVLVDVLKDKLKGQVMDLQHGGAFYSTRIRAAESYEDTAHSAVCIITAGVRQRPGESRLELMDRNAALFKGIIPPLVQYSPNTILLVVSNPVDLLTHLAWQMSGLPRERVIGSGTYLDSSRFRTLLAQRLGIDTASVQAMVLGEHGDSSFVYRSGITVGGVPLRTCFERMTDAASASTAFYDLVKGVHQQVVAAAYEVIKLKGYTNWAIGSAVGSIVTTIVHDRRKVLPITTHAGSLRGLESADVFLSLPCVLGRNGVVEVLQILPFMESDEKEDLQSSIEALQSTPKKAS

SEQ ID NO: 123 - protein, 320 aa, Spirochaeta africana
MIKNKIAIIGAGSVGATIAYNLSNRGLANEMVLVDVNREKAEAEVLDITHGMPLGSTANIYAAGYEACGDAEIAIITAGAKQRPDESRVQLMDRNVGIMRSMVGDLMASGFGGVILVVTNPVDVLTFVAYRESGLPAHQVIGSGTVIDSARLRTFLSRSCSINPQNVHGYVIGEHGDTSFPAWSNVTFGGVGVQEFCQDCDAGCGDDELRRQATEYVRQAAQTIIKAKGSTYYAVAQAVAIITQAVLRDERRILPITAVMSGFEDFREVAFSYPHFVGKNGIATDAGINGRLRYELTAEEQEQLRTSIRYIIGNTEQAGY

SEQ ID NO: 124 - protein, 350 aa, Rosa chinensis
MHKSTSASSLGPGGLDLTQAFFKPIHGAALPSSSNGQTKISVIGAGNVGMAIAQTILTQDLADELVLVDAIPDKLRGEMLDLQHAAAFLPRTKINASVDYAVTAGSDLCIVTAGARQIHGESRLNLLQRNVALFRKIIPPLAKYSPETILLIVSNPVDVLTYVAWKLSGFPSNRVVGSGTNLDSSRFRFLIADHLDVNAQDVQAYIVGEHGDSSVALWSSISVGGVPVLSFLKKQQIAYEKETLESIHKAVVDSAYEVISLKGYTSWAIGYSAAGLARSILRDQRSIHPVSVLAKGFYGVDGGDVFLSLPAQLGRSGVLGVTNVHLTDEEEQKLRDSAKTILEVQSQLGL

SEQ ID NO: 125 - protein, 319 aa, Fretibacterium fastidiosum
MQGKKRTVGIIGIGHVGAHVAYSLAVQGIADEIILVDRERKKADCEAQDVMDSVCYLPHRVEVRSGDFPDLKDCDVLVNSAGHIQLLATGNKSRLEEMDFTIRAVNGYVDRVMESGFDGVVINVTNPCDVVAWRFAELSGLPRGRVFGTGTGLDTARLRSALARQTGVDHKSICAYVMGEHGASQMVPWSSVSFGGRPLAEWERTDERFRFDREAIRKEARDAGWVVFSGKQCTEYGICSTAARMASVVLLDEKQILPVTTRLEGEYGESGIFIGVPAVVGAGGAEQVVEVPMSAEELAEFKGCCDDVRANMAHALEVR

SEQ ID NO: 126 - protein, 363 aa, Hypsibius dujardini
MAPPPAPGAVPATAAPSPATAAPSPAAAAPVGGDIRGKLMKDIQAPPETSLTKVTVVGVGQVGMAIAFSIVNRHLAGELCLVDVDEKKVKGELMDLQQGLQFAGNMKIQGSTNYDITAGSKLCIISAGARQKDGEDRRALLDRNIAIFKGIIPQLMKYSPDAVLCVVSNPVDVMTYLTWKISGLPPHRVFGSGCSLDSSRLRHYMAERLKIDVSSCHGFVIGEHGESSVVVWSGLNVAGVRLADIKPDIGTDKDSEKWVDVHRQVIDSATEIIKLKGYTSWAIGLCVSELCRAVIGNQRHVFSLSTMAKGYQGIDQEIFVSLPCVLSQNGVNAIVNLTLTATEKEKLKKSATELAELFKSAKL

SEQ ID NO: 127 - protein, 321 aa, Mycoplasma wenyonii
METVKIAVIGCGAVGSSFLYSAIHQGLASEYGLLDYNTEFARGQALDLEDAIPHFDFRPRIKVITDYKELKNYQFIVITAGRAQKEGETRLQMIRDNAVIMKGIAEQVKSSGFSGIVLICSNPVDVLTYIFQKVTGFDEKKVIGSGTVLDTNRLKVEVIKGMDVAPASLEGAFVLGEHGDSSLVTFSLMKVSGLSINRCEEVSYPNSPFCCSDYEEKLEKVVYKKAYEIISRKRATHYGIGVAMTKILKTIIYNTKEILPVSSILHGEYGLSDVAISVPTVVGSNGIERIAIIPLKEKEQNKLVASAKILQENIAKVRDLI

SEQ ID NO: 128 - protein, 319 aa, Thermotoga maritima
MKIGIVGLGRVGSSTAFALLMKGFAREMVLIDVDKKRAEGDALDLIHGTPFTRRANIYAGDYADLKGSDVVIVAAGVPQKPGETRLQLLGRNARVMKEIARNVSKYAPDSIVIVVTNPVDVLTYFFLKESGMDPRKVFGSGTVLDTARLRTLIAQHCGFSPRSVHVYVIGEHGDSEVPVWSGAMIGGIPLQNMCQICQKCDSKILENFAEKTKRAAYEIIERKGATHYAIALAVADIVESIFFDEKRVLTLSVYLEDYLGVKDLCISVPVTLGKHGVERILELNLNEEELEAFRKSASILKNAINEITAEENKHQNTSG

SEQ ID NO: 129 - protein, 310 aa, Verrucomicrobia subdivision 3 bacterium
MKVGVIGAGFVGSTGAYAMILQGVASEVVLVDINRELAQAQAEDMLHAIPFSPSARVEAGDYQDLRGARLVVLACGVGQKPGETRLQLLSRNAAVFRQVVPEVIKQAPEAVLMVVSNPVDLLTHIVTKLADLPAARIIGSGTILDTARFRALLAEEMAVTSHSVQAYVVGEHGDSEVLVWSSAQIGGLPLEDFAAQVKRPVTAEIEERIDKGVRQAAYRIIKGKAATYYGIGAGIARLARAIRDDERAVLTVSNAEIKPAQLPPVALSLPRVVGARGVLSTLRPTLSFQERDLLERSAHLLLANVQELGF

SEQ ID NO: 130 - protein, 312 aa, Smittium mucronatum
MNFTHRVSIIGGGGNVGAAVAFALVVMQLPVEILLLGASEKSARAQALDIRDAAHFSTAHCRAGTSEEVGCSDIIVITAGARQRPGEPRSNLIDRNYVILDSIIKKIQPIKPTAIILMVTNPVDVLTSLAQKLSGLPKSQVIGSGTFLDSGRLRNYLSRKLNVNSNSIHASMLGEHGDTQFVGWSVASIAGSPLLKHPLMANVDLAEIENAIAHQAYEIIEAKGSTYFGVGYHVAALIKCILTDGHKIYPVCNYNAKYDTYLSVPAILGSDGATPINLNLSDEEEVKLERCAESVNHSLGQVNEFAVHVNEE

SEQ ID NO: 131 - protein, 531 aa, Methylobacillus flagellatus
MRDMFTKDGRRFEKFSLEAEGLLLDYSKHRITDETLPLLFKLARDSKVEEWRDRMFAGEKINFTENRAVLHTALRNRSNTPVYVDGKDVMPDVNRVLAQMRKFSTSIRSGEWKGYSGKRITDVVNIGIGGSDLGPVMVCGALKPYAQAGLNAHFVSNIDGTHLAQTLERCDPETTLFIVASKTFTTQETMTNARSARSWFLQAAKDEAHVAKHFVAISTNADEVGKFGIDAANMFEFWDWVGGRYSLWSAIGLSIAIYIGMDHFEELLQGGYEIDRHFKNAPLEQNIPVIMALLGIWYNNFFGADSLAILPYDQGLARFPAYLQQADMESNGKFVARDGRIVQCTTGPIIWGEAGTNGQHAFYQLIHQGNRLIPCDFMMPLQSHYSMGKNGNEHHLILLANCFAQTSALMQGKTLDEAKAELVAQGLTGEALETLLPHKVFEGNRPSTTILFDKLTPKTLGKLIAIYEHKIFVQGIIWNINSFDQWGVEYGKQIAKKILPQLSEDQASTEYDSSTNGLMNYFKSRTQSSGT

SEQ ID NO: 132 - protein, 209 aa, Methylobacillus flagellatus
MSTLDLANHGPVIPVIVINKVEDAVPMAEALLEGGIKVLEVTLRTPVALQAMEAIAKAVPDAIVGAGTVRNIKDAQNCKDVGCQFAVSPGYTSELGRAAREMGLPLLPGVSTGSEIMQANADDYYFLKLFPAVAVGGINLLKGFAGPFGDVKFCPTGGLTVESAPQFLALPNVVVCGGTWLTPGDAVARKDWAHITKLAREASAIKAAA

SEQ ID NO: 133 - protein, 226 aa, Pseudomonas putida
MTTLERPQPKLSMADKAARIDAICEKARILPVITIAREEDILPLADALAAGGIRTLEVTLRSQHGLKAIQVLREQRPELCVGAGTVLDRSMFAAVEAAGAQFVVTPGITEDILEAGVDSEIPLLPGISTPSEIMMGYALGYRRFKLFPAEISGGVAAIKAFGGPFGDIRFCPTGGVNPANVRNYMALPNVMCVGTGWMLDSSWIKNGDWARIEACSAEAIALLDAN

SEQ ID NO: 134 - protein, 213 aa, Escherichia coli
MKNWKTSAESILTTGPVVPVIVVKKLEHAVPMAKALVAGGVRVLEVTLRTECAVDAIRAIAKEVPEAIVGAGTVLNPQQLAEVTEAGAQFAISPGLTEPLLKAATEGTIPLIPGISTVSELMLGMDYGLKEFKFFPAEANGGVKALQAIAGPFSQVRFCPTGGISPANYRDYLALKSVLCIGGSWLVPADALEAGDYDRITKLAREAVEGAKL

SEQ ID NO: 135 - protein, 228 aa, Methylobacillus flagellatus
MAKPLVQMALDSLDFDQTVALATTVAPHVDILEIGTPCIKYNGIKLLETLRAKFPNNKILVDLKTMDAGFYEAEPFYKAGADIVTVLGTADIGTIKGVIDVANKYGKKAQVDLINVTDKAARTKEVAKLGAHIIGVHTGLDQQAAGQTPFADLNLVSSLNLGVDISVAGGVKATTAKQVVDAGATIVVAGAAIYGAADPAAAAAEISAAAKGTQSSGGLFGWLKKLFS

SEQ ID NO: 136 - protein, 181 aa, Methylobacillus flagellatus
MNKYQELVVNKLTNVINNTAEGYDDKILSMVDAAGRTFLGGAGRSLLVSRFFAMRLVHAGYQVSMVGEVVTPSIQAGDLFIVISGSGSTETLMPLVRKAKSQGAKVIVISMKAQSPMAELADLVVPIGGNDAHAFDKTHGMPMGTIFELSTLWFLEATIAKLIDQKGLTEEGMRAIHANLE

SEQ ID NO: 137 - DNA, 1002 bp, Methylobacillus flagellatus
atgcgcatcgtctttttcagcacccaggtatatgaccgggaaagttttctggccctccccaggctccagaatgccgagttcattttccaacagcccaaactcacgttggatactgccgtgcttgccacaggcgcggaagtcgtctgtgccttcatcaatgacgacctgtccgcgcctgtgctggagagactggcagccaacggtaccaagctgattgcactgcgctccgcaggctacaaccatatcgacctggaggctgcgcaaagactcaacctggcagtggtgcgcgtgcccgcctattcgccccatgccattgcggaacataccgtcgcattgatcctggccctcaatagacacctgacgcgcgcctacaaccgtacccgcgagggtgatttcagcctgcgcggcttgacagggttcgacctagtccacaagacagtaggcatcatcggcaccggacagatcggtgcagcttttgcccgcatcatggcaggtttcggctgcaggatactggcttacgatccctaccccaacccggaagtcattgcgctcggcgccagctacctcgaactcgatacgctgttggcgcaatcccacatcgtcagcctgcattgcccgttgagccctgccacccaccatctcatcaatgccggttcgctcagccgcatgcagccaggcagcatgctcatcaacaccagccgcggcgcactcgtggatacgccggccgtgatcgaagcgctgaagagcggacacctcggctatcttgggctggacgtctatgaagaagaagcagacctgtttttcgaggacctatccgactttccgttgcaggatgacgtactggcgcggctgctgacctttcccaacgtcatcatcactgcccaccaggcgtttctcacacgcgaagcgctcaatgccattgccagcaccacgttagacaatatcagcgcctgggcagcaggccaccctcagaacctggtcaggctggaaacaggaagctga

SEQ ID NO: 138 - DNA, 1002 bp, Methylobacillus sp
atgcgcatcgtctttttcagcacccaggtatatgaccgggaaagttttctggccctccccaggctccagaatgccgagttcattttccaacagcccaaactcacgttggatactgccgtgcttgccacaggcgcggaagtcgtctgtgccttcatcaatgacgacctgtccgcgcccgtgctggagagactggcagccagcggcaccaagctgattgcactgcgctccgcaggctacaaccatatcgacctggaggctgcgcaaagactcaacctggccgtggtgcgcgtgcccgcctattcgccccatgccattgcggaacataccgtcgcattgattctggccctcaatagacacctgacgcgcgcctacaaccgtacccgcgagggtgatttcagcctgcgcggcttgacagggttcgacctagtccacaagacagtaggcatcatcggcaccggacagatcggtgcagcttttgcccgcatcatggcaggtttcggctgcaggatactggcttacgatccctaccccaacccggaagtcattgcgctcggcgccagctacctcgaactcgatacgctgttggcgcaatcccacatcgttagcctgcattgcccgttgagccctgccacccaccatctcatcaatgccggttcgctcagccgcatgcagccaggcagcatgctcatcaacaccagccgcggcgcactcgtggatacgccggccgtgatcgaagcgctgaagagcggacacctcggctatcttgggctggacgtctatgaagaagaagcagacctgtttttcgaggacctatccgactttccgttgcaggatgacgtactggcgcggctgctgacctttcccaacgtcatcatcactgcccaccaggcgtttctcacacgcgaagcgctcaatgccattgccagcaccacgttagacaatatcagcgcctgggcagcaggccaccctcagaacctggtcaggctggaaacaggaagctga

SEQ ID NO: 139 - DNA, 996 bp, Methylobacillus rhizosphaerae
atgcgtatcgtctttttcagcacccaggtatatgacaaggaaagttttctggctttccccaggctccagaacgctgaattcatcttccagcaacccaagctgacggtagataccgccgtgcttgccgatggagctgaagtcgtctgcgcattcatcaatgacgacctgtcagcaccagtgctggagaaactggcggccaacggcacaaaactgatcgcattgcgctcagcaggctacaaccatatcgacctggaagccgcgcaacgacttaacctggctgtcgtgcgcgtaccatcttattcaccacatgccattgccgagcataccgtcgccttgatccttgcgctcaacaggcatttgacgcgtgcctacaaccgcacgcgcgaaggtgatttcagcctgcgcggattgacaggtttcgatctggtcaacaagacggtaggcgttgtcggcacagggcaaatcggcgcaacgtttgcgcgcatcatggcaggtttcggttgcaagatactggcctatgatccgtatcccaacccgcaagtcactgcgctgggagcaagttaccttgagctcgatacgctattggcgcaatcccatatcgtcagcctgcattgcccgctgagtcccgaaacccatcacctgatcaatgccagctcgctcagccgcatgcagcagggcagcatgctcatcaacaccagccgtggcgcattggtggacacgcctgccgtcattgaggcattgaaacgtgggcacttgggctacctgggcctggatgtgtatgaagaagaggcagatttgttcttcgaggacctatccgattttcccttgcaggacgatgtgctggcacgcctgctgaccttccccaacgtcatcatcactgcgcaccaggcttttctcacgcgcgaagcgcttgatgcgattgcgggcaccacgcttgccaacatcgacgcttgggcggcaggcaggccgcaaaacctggtcaggctggaaacatga

SEQ ID NO: 140 - DNA, 996 bp, Methylobacillus methanolivorans
atgcgtatcgttttcttcagcacccaggcctatgacagggagagctttctcgcatttcccaagccccagaatgcggaattcatttttcagcaacccaagctcactacagataccgcggtgcttgccgctggagcggaagtcgtctgtgctttcatcaatgatgatttatctgctccggtgctagagaaattagcctctggcggcaccaagctgattgcacttcgctcggcaggctataatcatattgacctggaagccgcgcagaaactagggctggcagtcgcccgagtaccatcgtattcaccacatgccattgccgaacataccgtagcgctgatcctcgccttgaaccggcacctgacacgtgcctacaaccgtacgcgcgaaggcgacttcagcctgcgcggcctaaccggctttgatctcgtcaacaagaccgtaggcgtgattggcaccgggcagataggcgcagcatttgcccgcatcatggcgggatttggctgcaaggtgctagcctacgatccctaccccaacccggaggttatcgcgctaggagcatgctatctcgatcttgatacattgctggcacaatcgcatattgtcagcctgcactgcccgctgagcccagcaacgcatcacctgatcaatgctaactcactcgcccacatgcggcgtggcagtatgctgatcaataccagtcgcggcgcattagtggatacacctgcagtgattgatgccttgaaaagcggccatctaggttacctggggctagatgtttatgaagaagaagcggacctgttcttcgaggatttatcggattttccgttgcaagacgacgtactggcgcgcctgctgaccttccccaacgtcatcatcactgcgcatcaggcgttcctcacacgtgaagcgctggatgccattgccagcaccaccttgtccaatatcgagcaatgggcaacgggcacgccgcaaaacctggtcaggctggaagcatga

SEQ ID NO: 141 - DNA, 996 bp, Methylobacillus arboreus
atgcgcatcgtctttttcagtacccaggtttatgatcgcgagagctttctcgcattacccaggtctccaaatacggaattcgtattccagcaacccaagctaacagcagatacagcggtgcttgctgcgggcgcagaagttgtctgtgcctttatcaatgacgatttgtctgccccggtattggaaacactggcggcgggtggtaccaaactgatcgcgcttcgctcggccggctacaaccatattgatcttgaggccgcacacacactcaagctagaagtcgtccgcgtgccagcctattcgccacatgccattgccgagcataccgtggcgcttatcctcgcactcaatcgccacctcacccgcgcctacaaccgtacgcgcgaaggcgatttcagcctgcgtggtctcactggctttgatctggtcaacaagaccgtaggtgtcattggtaccgggcaaattgggacggcgtttgccaggatcatggctgggttcggctgcaagatacttgcttacgatccctatcccaacccggaggtagaagccctgggggtgcgttacctggaactggatgagttgctggcgcaatcgcagatcgtgagcctgcactgcccgctgagcccggccacttaccacttgatcaacgaaagtgcgcttaaccgcatgcagcgtggcagcatgctcatcaataccagtcgtggcgcactggtagacacgcctaccgtgattgacgctttaaagagcgggcacctgggctatctgggcctggatgtctatgaagaggaagcggatttattctttgaggatttgtcggatttcccgttgcaggacgatgtgcttgcaaggttactgacctttcccaacgtcatcatcaccgcgcatcaagcttttctcacacatgaagcgctggatgccattgctagcaccacccttgacaacatcgttgcctgggctgaaggtaggccacaaaacttggtgaagctggaaacatga

SEQ ID NO: 142 - DNA, 996 bp, Methylobacillus caricis
atgcgtatcgtttttttcagcacccaggcttatgaccgtgaaagctttctcgagcacgacaaacccaacgatgcagaatttgtattccagcaacccaaactgactttggaaacggcggttcttgccgctggggctgaggtagtttgcgcattcatcaatgacgatctgtccgctcccgttctggaacaacttgcagccaacggtacacgcttgatcgccctgcgttcagccgggtacaaccatattgacctggaagcagccacacgacttggcctggcagtagcacgagtaccatcctattcgccgcatgccattgcagaacatactgtcgccttgatactggcactcaaccgccacctgacacgggcttataatcgcacgagggagggcgacttcagcctgcgcggcctcacgggcttcgacctggtaaacaagacagtgggtatcatcggtacgggccagataggagctgcatttgccaagatcatggcagggtttggctgcaaactgctggcatatgatccttatcccaaccctaaggtagtaaagttgggtgcgcaatatctggagctggatgaactttttggccaggcccagattgtcagcctgcattgtccattgagtcccagcacttatcacctgatcaatgcgagcacactaggccggatgcagtctggcagcatgctcatcaataccagccgtggcgcactggtggatactcctgcagtaattgaggcgctgaaaagcggccacctgggttacctgggcctggatgtctatgaagaagaggccgatctgtttttcgaggatttgtcagattttcctttgcaggatgatgtgctggcacgcctgctgacttttcctaacgtcatcatcactgcccatcaggcattcctcacgcgcgaggccctgaatgcgattgcaagcacaaccctagccaacatcagcgcatgggccgagggatcaccgcaaaacctggtcaacatagaaggatag

SEQ ID NO: 143 - DNA, 996 bp, Methylobacillus gramineus
atgcgtatcgtttttttcagcacccagacttatgaccgtgaaagttttctcgggcttgataagccgacaggcgcagaatttgtatttcagcaaccgaaactgaccgtcgatactgcggttcttgccgccggcgcagaggtagtgtgtgcgttcatcaatgatgatctgtccgccccagtactggatcagctggcagccacaggcacacgcttgattgcattgcgctcggccgggtacaaccatatcgacctggaagcggcacagcgcctgggcctggtagtgacacgcgtaccgtcttattcgcccaatgccattgcagaacataccatcgccctgatactggcactcaatcggcacctgacgcgtgcctataaccggacgcgagaaggagatttcaacctcagaggcctcacaggctttgatctggccaacaagacggtggggattataggtaccgggcagataggtgcagccttcgcacggatcatggccggatttggctgcaaactactggcgtatgacccttaccccaaccctgaagtgaccgcactcggtgcggaatacctgccgctggatgcgttattcagccgggcccagattgtcagcctgcactgtcctttaagccccaacacctttcatctgatcaatgctgagacactcaaccgcatgcaacgcggcagtatgctgatcaataccagccgtggtgcattggtcgatacgccagccgtgatcgaggcattgaaaagcggtcacctgggctatcttggcctggatgtatatgaggaggaggcagacctgttttttgaggatctttccgattttcccttgcaagatgatgtcctggcacgtctgctgacttttcccaacgtcatcatcaccgcacatcaggctttcctcacacgtgaagcactacatgcgattgcaagtaccaccctggccaatatcagcgcctgggccgcaggatccccatgcaatctggtaaaggcagaagcttga

SEQ ID NO: 144 - DNA, 993 bp, Methylobacillus glycogenes
atgcaaatcgtttttttcagcacccaggcctacgaccgtgaaagttttctctcgcagcccgcattgagtgactgcgagctggtgttccagcaacccaaactgactgtggataccgccgtgctcgccgcaggggccgaggtggtgtgtgcgttcatcaatgatgatctttccgcagctgtactggaaaagctggccgcaggcggcacacgtttgattgcactgcgctcggcaggctataaccatattgatcttgaagccgccaagcgcctggcgctggccgtggtgcacgtgccctcatactcgccccacgcgattgccgagcacaccatcgcactgatattggcgctcaaccgtcacctcaaccgagcttataaccgcacccgcgaaggcgatttcagcctgcgcgggctgactggctttgatctggtgaacaagacggtgggcattataggcaccgggcaaataggcgcggctttcgcccgcatcatggcgggctttggttgcaggctgctggcttatgacccttaccccaatcctgaggtaatagcactgggggccgagtatctgccactggaacagttgtttccgcaagcacatatcgtcagcctgcactgtccgctaagcccggccacgcatcatttgattaacccccagaccctggccctgatgcaaaaaggcagcatgctgatcaataccagccgcggcgccctggtcgacacgcccgccgtgattgaggcattaaaaactggccatctgggccacttggggctggatgtctatgaagaagaagcagacttgttcttctctgatctttccgactatccgctgcaggatgatgtattggccagactgttgaccttccccaatgtcatcatcaccgcgcatcaggcatttttgacgcgcgaggccctggctgggattgccagcaccacgctgctgaatgttgccgcctggcggcgtggtcagccgcagaatctggtgcagccaggctag

SEQ ID NO: 145 - DNA, 990 bp, Escherichia coli
atgaaactcgccgtttatagcacaaaacagtacgacaagaagtacctgcaacaggtgaacgagtcctttggctttgagctggaattttttgactttctgctgacggaaaaaaccgctaaaactgccaatggctgcgaagcggtatgtattttcgtaaacgatgacggcagccgcccggtgctggaagagctgaaaaagcacggcgttaaatatatcgccctgcgctgtgccggtttcaataacgtcgaccttgacgcggcaaaagaactggggctgaaagtagtccgtgttccagcctatgatccagaggccgttgctgaacacgccatcggtatgatgatgacgctgaaccgccgtattcaccgcgcgtatcagcgtacccgtgatgctaacttctctctggaaggtctgaccggctttactatgtatggcaaaacggcaggcgttatcggtaccggtaaaatcggtgtggcgatgctgcgcattctgaaaggttttggtatgcgtctgctggcgttcgatccgtatccaagtgcagcggcgctggaactcggtgtggagtatgtcgatctgccaaccctgttctctgaatcagacgttatctctctgcactgcccgctgacaccggaaaactatcatctgttgaacgaagccgccttcgaacagatgaaaaatggcgtgatgatcgtcaataccagtcgcggtgcattgattgattctcaggcagcaattgaagcgctgaaaaatcagaaaattggttcgttgggtatggacgtgtatgagaacgaacgcgatctattctttgaagataaatccaacgacgtgatccaggatgacgtattccgtcgcctgtctgcctgccacaacgtgctgtttaccgggcaccaggcattcctgacagcagaagctctgaccagtatttctcagactacgctgcaaaacttaagcaatctggaaaaaggcgaaacctgcccgaacgaactggtttaa

SEQ ID NO: 146 - DNA, 1191 bp, Escherichia coli
atgattatttccgcagccagcgattatcgcgccgcagcgcaacgcattctgccgccgttcctgttccactatatggatggtggtgcatattctgaatacacgctgcgccgcaacgtggaagatttgtcagaagtggcgctgcgccagcgtattctgaaaaacatgtccgacttaagcctggaaacgacgctgtttaatgagaaattgtcgatgccggtggcactggctccggtgggtttgtgtggcatgtatgcgcgtcgtggcgaagttcaggcagccaaagcggcggacgcgcatggtattccgtttactctctcgacggtttccgtttgcccgattgaagaagtcgcgccagccatcaagcgcccaatgtggttccagctttatgtactgcgcgatcgcggctttatgcgtaacgcgctggagcgagcaaaagcagcgggttgttcgacgctggttttcaccgtggatatgccgacaccgggcgcacgctaccgtgatgcgcattcaggtatgagcggcccgaacgcggcaatgcgccgctacttgcaagcggtgacacatccgcaatgggcgtgggatgtgggcctgaacggtcgtccacatgatttaggtaatatctcagcttatctcggcaaaccgaccggactggaagattacatcggctggctggggaataacttcgatccgtccatctcatggaaagaccttgaatggatccgcgatttctgggatggcccgatggtgatcaaagggatcctcgatccggaagatgcgcgcgatgcagtacgttttggtgctgatggaattgtggtttctaaccacggtggccgccagctggacggtgtactctcttccgcccgtgcactgcctgctattgcagatgcggtgaaaggtgatatagccattctggcggatagcggaattcgtaacgggcttgatgtcgtgcgtatgattgcgctcggtgccgacaccgtactgctgggtcgtgctttcttgtatgcgctggcaacagcgggccaggcgggtgtagctaacctgctaaatctgatcgaaaaagagatgaaagtggcgatgacgctgactggcgcgaaatcgatcagcgaaattacgcaagattcgctggtgcaggggctgggtaaagagttgcctgcggcactggctcccatggcgaaagggaatgcggcatag

SEQ ID NO: 147 - DNA, 1008 bp, Fusobacterium nucleatum
atgcaaaaaactaagataatattttttgatataaaagattatgataaagaattttttaagaaatatggagcagattataattttgaaatgacttttttaaaagttagattgacagaggaaacagctaacttaacaaaaggttatgatgttgtttgtggttttgctaatgataatataaataaagaaactattgatattatggctgaaaatgggataaaacttttagctatgagatgtgcaggttttaataatgtatctttaaaagatgtcaatgaaagatttaaagtggttagggttcctgcttattcacctcatgcaatagcagaatatacagtgggacttatcttagcagtcaatagaaaaattaacaaagcatatgttcgtacaagagaaggaaatttttctataaatggattaatgggaattgatttatatgaaaaaacagcagggattataggaactggaaaaattgggcaaattttaataaaaatattaagaggttttgatatgaaagttattgcttatgacctattcccaaatcaaaaagttgcagatgagcttggttttgaatatgtaagtttagatgaactttatgcaaactcagatattatttctttaaactgtcctcttacaaaagatacaaaatatatgattaatagaagatctatgctaaagatgaaagacggggttatcttagtaaatacaggtagaggaatgttaattgattctgctgatttagtcgaagcattaaaagataaaaaaattggagctgttgctcttgatgtatatgaagaagaagaaaattatttctttgaagataaatctacacaagttatagaagatgatattttgggaagacttttatctttctataatgttcttattacatcacaccaagcatattttacaaaagaagcagttggagcaattacagttactactttaaataatataaaagattttgttgaaggtagaccattagtaaatgaagttccacaaaatcaataa

SEQ ID NO: 148 - DNA, 990 bp, Pseudomonas aeruginosa
atgcgcatcctgttcttcagcagccaggcctacgacagcgagagcttccaggccagcaaccaccggcacggcttcgaactgcacttccagcaggcccacctgcaggcggacacggcggtcctcgcccagggcttcgaagtagtctgcgccttcgtcaacgacgacctctcgcggccggtgctggaacgcctggcggccggcggcacgcgcctggtcgccctgcgctcggccggctacaaccacgtcgacctggccgccgccgaagcgctcggcctgccggtggtgcacgtcccggcctattcgccgcacgctgtcgccgagcacgcggtcggcctgatcctgacgctcaaccggcgcctgcaccgcgcctacaaccggacccgcgagggcgatttctcgctgcatgggctgaccggcttcgacctccacggcaaacgcgtcggagtgatcggcaccggacagatcggcgagaccttcgcccgcatcatggccggcttcggctgcgagctgctggcctacgatccttatcccaatccgcgcatccaagcactcggcggccgctacctggcgctcgacgccctgctcgccgagtccgacatcgtcagcctgcattgcccgctgaccgccgacacccgccacctcatcgacgcgcagcgcctggcgacgatgaaacccggcgcgatgctgatcaataccggccgtggcgccctggtgaacgccgcggcgctgatcgaggcgctgaagagcggacaactgggctacctcggcctcgatgtctatgaagaggaagcggatatctttttcgaggatcgctccgaccagcccctgcaggatgacgtgctggcacgcctgctgagcttccccaacgtggtggtgacggcccaccaggccttccttacccgcgaggccctggcggcgatcgccgacaccaccctggacaacatcgccgcctggcaggacgggacgccgcgcaatcgggtccgggcctga

SEQ ID NO: 149 - DNA, 963 bp, Pedicoccus sp
atgtccaagatccagaatcatcagaaggtggtcctggttggtgacggtgccgtcggcagcagctatgctttcgcgatggcgcagcagggcatcgcggaagaatttgtcattgtggatgtggtgaaagaccgcaccgtgggcgacgcgctcgatctcgaagatgccaccccgttcaccgcgcctaaaaatatctacagcggcgaatattccgactgcaaggatgcggatctcgtcgtgattaccgccggcgccccgcagaagccgggcgaaacgcgcctcgacctcgtgaataaaaatctgaatatcctcagcacgattgtgaaaccggtggtggacagcggttttgacggcatttttctggtggccgccaatccggtggatattctcacctacgcgacgtggaagtttagcggctttcctaaggaaaaagtgattggcagcggcatctccctcgatagcgcgcgcctccgcgtggccctcggcaaaaagtttaatgtgtcgcctgacagcgtggatgcgtacattatgggcgaacatggcgacagcgaatttgccgcctacagcaccgccagcattggcacgaaaccgttgctcgatattgccaaggaagaaggtgtgagcaccgacgaactggccgaaattgaagacagcgtgcgcaataaggcctacgaaattattaataaaaaaggcgccacgttttacggcgtgggcaccgccttgatgcgcatcagcaaggccattttgcgcgacgaaaacgccgtcttgcctgtgggcgcctacatggacggtgaatatggcttgaacgacatttacattggcacgcctgccgtgatcaatggtcagggcttgaatcgcgtgattgaaagcccgctcagcgatgacgaaatgaaaaaaatgacggatagcgccacgacgttgaagaaggtgctcacggatggcttgaaggccctcgaagaaaagtga

SEQ ID NO: 150 - DNA, 1596 bp, Methylobacillus flagellatus
atgcgggacatgtttaccaaggatgggcgcagattcgaaaagttctccctggaagcggaaggcctgttgctggactactccaagcaccgcatcacggatgaaaccctgccgctactgttcaagctcgcgcgcgactccaaggtcgaggaatggcgtgaccgcatgttcgcgggcgagaagatcaactttacggaaaaccgtgctgtactacataccgccttgcgcaaccgtagcaatacgcccgtatatgtggatggcaaggatgtcatgcccgacgtcaaccgcgtactggcccagatgcgtaaattcagcaccagcatccgctctggggaatggaaaggctactcaggcaagcgcattaccgatgtcgtcaacatcggcatcggcggctcggacctcggcccagtcatggtgtgcggggcgctcaagccttatgcccaggctgggctgaacgcgcatttcgtgtccaatatcgacggcacccacctcgcccagaccttggaacgctgcgatccggaaaccactttgttcatcgtcgcttccaagactttcaccacccaggagaccatgaccaatgcgcgctctgcccgcagctggttcctgcaggcagccaaggatgaggcgcacgttgcaaaacacttcgtcgcgatttccaccaatgcggacgaagtcggcaagttcggcatcgatgccgccaatatgttcgaattctgggattgggtaggcgggcgctattccctatggtccgcaatcggcctctcgattgccatctacatcggcatggatcatttcgaggagttgctgcaaggcggctacgaaatcgaccggcatttcaagaatgcgccgctggagcagaacattcccgtgatcatggcgctgctgggcatctggtacaacaatttcttcggtgcagacagcctcgccatcctgccttacgaccaggggcttgcccgcttccctgcctacctgcagcaagccgatatggaaagtaacggcaagtttgtcgcccgagacggccgcattgtgcaatgcaccaccggccccatcatctggggcgaggctggcaccaacggccagcatgcgttctaccaactgatccaccagggcaaccgtctgatcccctgcgatttcatgatgccactgcagagccactacagcatgggcaaaaatggcaatgaacaccacctcatcctgctggccaattgcttcgcgcaaaccagcgcgctcatgcagggcaagacactggatgaagccaaggccgaactggttgcgcaaggattgactggtgaagcgctggaaaccctgctgccgcacaaagtctttgagggaaaccgcccaagcaccaccatcctgttcgacaagctgacgccaaagaccctgggcaagctgatcgcgatctacgaacacaagatattcgtgcaaggcatcatctggaacatcaactcctttgaccaatggggcgtagaatacggcaagcaaattgccaagaaaatcctgcctcagctgagcgaagatcaggcatcgactgagtacgacagctcgaccaatggcctgatgaattacttcaaatcgcggacacaatcctcgggcacctaa

SEQ ID NO: 151 - DNA, 630 bp, Methylobacillus flagellatus
atgagcacactcgatttagccaaccatggcccagtcatcccggtcattgtcatcaacaaagtggaagacgcggtgccgatggcagaagctttgctcgaaggtggtatcaaggtactggaagtgaccttgcgcacgccagtggccttgcaggccatggaggccatcgccaaggccgtgcctgatgccatcgtgggtgccgggactgtgcgcaacatcaaggatgcgcaaaactgcaaggatgttggctgtcaattcgccgttagcccaggctataccagtgaactgggccgtgctgcgcgtgaaatggggttgccattgctgcctggcgtatcgaccggtagcgagatcatgcaagcaaatgccgatgattactatttcctcaagctgttcccggctgttgctgtgggtggcattaacctactcaagggctttgccggcccgttcggcgatgtcaagttctgccctacgggcgggctaacggtagaatcggctccccagtttctggcgttgcctaacgtcgtggtttgcggcggcacctggctcacgcctggcgatgccgtggcgcgcaaggattgggcgcatatcaccaagctggcgcgcgaggccagtgcgatcaaggctgcagcctaa

SEQ ID NO: 152 - DNA, 681 bp, Pseudomonas putida
atgaccaccctcgaacgcccacagccaaagctctcgatggccgacaaggccgcccggatcgatgccatctgcgaaaaggcgcgcatcctgccggtcattaccatcgcccgtgaggaagacatcctgccgctggccgatgccctggccgccggcggtatccgtaccctggaagtgaccctgcgttcccagcatgggctcaaggccatccaggtgctgcgtgagcagcgcccggagttgtgcgttggggcaggcaccgtactggatcgcagcatgttcgccgctgtcgaggctgcgggcgcgcagttcgtcgtcaccccgggcattacccaggacattctcgaagcgggcgtggacagcgaaatcccgctgctgccaggcatcagtacgccctctgaaatcatgatgggctatgccctgggctaccgcaggttcaagttgttcccggcggaaatcagcggcggcgtggcggcgatcaaggcctttggcggcccgttcggcgatattcgcttttgcccaaccggcggcgttaacccggccaatgtacgtaactacatggcattgcccaacgtgatgtgcgtgggcggaacctggatgctcgacagcagctggatcaagaacggcgactgggcgcggatcgaagcgtgcagcgcggaggcgatggcactgttggacgccaactga

SEQ ID NO: 153 - DNA, 642 bp, Escherichia coli
atgaaaaactggaaaacaagtgcagaatcaatcctgaccaccggcccggttgtaccggttatcgtggtaaaaaaactggaacacgcggtgccgatggcaaaagcgttggttgctggtggggtgcgcgttctggaagtgactctgcgtaccgagtgtgcagttgacgctatccgtgctatcgccaaagaagtgcctgaagcgattgtgggtgccggtacggtgctgaatccacagcagctggcagaagtcactgaagcgggtgcacagttcgcaattagcccgggtctgaccgagccgctgctgaaagctgctaccgaagggactattcctctgattccggggatcagcactgtttccgaactgatgctgggtatggactacggtttgaaagagttcaaattcttcccggctgaagctaacggcggcgtgaaagccctgcaggcgatcgcgggtccgttctcccaggtccgtttctgcccgacgggtggtatttctccggctaactaccgtgactacctggcgctgaaaagcgtgctgtgcatcggtggttcctggctggttccggcagatgcgctggaagcgggcgattacgaccgcattactaagctggcgcgtgaagctgtagaaggcgctaagctgtaa

SEQ ID NO: 154 - DNA, 687 bp, Methylobacillus flagellatus
gtggcaaaaccattagttcaaatggcattagattcactagatttcgatcagactgtagcgcttgctacgactgttgcaccacatgttgatattcttgaaatcggtactccttgtatcaagtacaacggtatcaagttgctggagactctccgcgcaaagttccctaacaacaagatcctggttgacctgaagaccatggatgctggtttttacgaagcagagcctttctacaaggcaggtgccgacatcgtgaccgtgctcggcactgctgacattggcacgatcaaaggcgtcattgatgttgccaacaaatacggcaagaaggctcaagtcgacctgatcaacgtgactgacaaggctgcacgcaccaaggaagtggccaagctcggcgctcacatcattggcgttcacactggtttggatcaacaggctgctggtcagacaccgtttgccgatctcaaccttgtttccagcctgaacctgggtgttgacatttccgtagctggtggcgtgaaggcgactaccgccaaacaagtggttgatgcaggtgccacaattgttgttgctggtgcggctatctatggtgctgccgatcctgctgctgctgctgctgaaatcagcgctgcggccaagggtacacaaagcagtggtggcctgtttggctggctgaagaaactgttcagctaa

SEQ ID NO: 155 - DNA, 546 bp, Methylobacillus flagellatus
atgaataaatatcaagagctcgtggtcaacaagctgaccaatgtaatcaataacacagcagaaggctatgatgacaagatcctgagcatggtggatgctgccggtcgtaccttccttggtggtgctggtcgttccctgctggtttcccgcttcttcgccatgcgtctcgtccatgcaggctatcaagtcagcatggtgggtgaggttgtcactccgagcatccaggctggcgaccttttcattgtgatctccggttcgggaagcacggaaaccctgatgcccttggtcaggaaggccaagagccagggcgcaaaggtcatcgtgatctccatgaaggcgcagtccccaatggcggagctggcagacctagtggtgccgatcggtggcaacgatgcgcatgcattcgacaagacacatggcatgcctatgggcactattttcgagctgtctacgctctggttcctggaagctacgattgccaagttgatagatcaaaaaggcctgacagaagaaggcatgcgtgcaattcacgccaatcttgaataa

SEQ ID NO: 156 - protein, 693 aa, Methylobacillus flagellatus
MLPVKLTPEYFINRELGILAFNRRVLAQAEDERVPLLERLKFLCIFSSNMDEFFEVRVAGLKNQIKYNSPHVGADGMLPKQALAKISKLAHEMVDHQYKILNEIVLPQLAAQEIRFIRRGDWNEVQREWIATYFFRELMPILTPIGLDPAHPFPRVLNKSLNFAVELEGKDAFGRNSGVAIVQAPRALPRVIRLPRDIAGCDHGFVFLSSILHAHVNELFSGMTVKGCYQFRVTRDSELTLDDEETKDLRLALQGELTHRQYGDAVRLEVADSCPAEMSAFLLGQFGLGQDDLYQVNGLVNLVRLMQIPDSVDRPDLKYPHYTPSLPRELDKDQDIFKAIRKQDILLHHPFQSFNPVVEFIKQAAEDPQVLAIKQTFYRTSADSTLMTSLIDAAQRGKEVTVVVELLARFDEEANINWAAKLENAGAHVVYGVVGHKTHAKMAMVVRRDEDKLRRYVHIATGNYHQRTARLYTDFGLLTCQEEISEDVNDVFAQLTGLGKASKLRHLWQSPFTLHQRTVKAIQNEAEIARSGKKARIIAKMNALLDPDVIRALYDASCAGVQIDLIVRGVCALRPGIPGISENIRVRSIVGRFLEHTRIFYFYDDGAEHIYLSSADWMYRNFFRRIEVCFPLLDAKVKKRVFKEGLEPYLKDNSNAWEMQSDGHYERKASRRASFAAQQFLMAEHGQEILPES

SEQ ID NO: 157 - DNA, 2082 bp, Methylobacillus flagellatus
atgttgcccgtcaaattgactcccgagtatttcatcaatcgcgagctaggcattctcgccttcaaccgtcgcgtattggcccaagctgaggacgaacgcgtacccctgcttgaacgcctcaagttcctctgcattttcagcagcaatatggatgagttcttcgaggtgcgcgtagcaggcctcaagaaccagatcaaatacaactcgccgcatgtaggcgccgacggcatgctgcccaagcaggcgctcgccaagatcagcaagctggcgcatgaaatggtggatcaccagtacaagatcctcaatgaaatcgtactcccacagctggcagcccaggaaatccgctttatccgccgcggtgactggaacgaggtccagcgcgagtggattgctacttacttcttccgcgagttgatgcccattctcaccccgatcgggctggatccagcacacccgttccctcgcgtactgaacaaaagcctgaactttgccgtcgagctggaaggcaaggacgccttcgggcgcaattcgggcgtcgccatcgtgcaggcgccgcgcgcgctgccgcgcgtcatccgcctgccgcgcgacattgccggctgcgaccatggtttcgtattcctgtcatccatcctgcacgcgcatgttaacgaactgttctccggcatgacggtaaaaggttgctaccagttccgcgtcacgcgcgatagcgagttgaccttggatgatgaagagaccaaggacttgcgcctcgccctgcaaggtgagctgactcaccgtcaatacggcgatgccgtacgcctggaagtagccgacagctgcccggcggaaatgtccgcctttttactgggtcaatttggcctgggccaggacgacctctaccaggtcaatggtctggtcaacctcgttcggctgatgcagatcccggacagcgtggaccgcccggacctgaagtatccgcattacacgcccagcctgccacgggagctggataaggaccaggacatcttcaaggccatccgcaagcaggatatcctgctgcatcatccattccagtcgttcaatccggtagtagaattcatcaagcaggctgcggaggatccgcaagtgttggccatcaagcagacgttctaccgcaccagcgcagactccacactgatgacatccctgattgacgccgcacagcgcggcaaggaagtcaccgtggtggtggagctgttggcacgctttgatgaagaagccaatatcaactgggcagccaagctggaaaatgccggcgctcacgtcgtgtatggcgtggtggggcacaagacccatgccaagatggccatggtggtgcggcgcgatgaagacaagctgcggcgttatgtgcatattgccaccggcaactaccaccagcgtaccgcgcgcctgtataccgacttcggcctgctcacctgccaggaagaaatcagcgaggatgtgaatgacgtcttcgcccagctgacgggcctgggcaaggctagcaagctgcgccatctctggcagtcgccgttcaccttgcaccagcgcacggtcaaggcaatccagaatgaagcggaaattgccaggtcgggcaagaaggcccgcatcattgccaagatgaatgccctactcgatcccgacgtgatccgagccttgtacgatgcctcctgcgccggcgtgcaaatcgacctcatcgtgcgcggcgtctgcgccctccgcccaggcattccgggcatatcggagaatatccgggtgcgttccatcgtgggacgatttctcgagcacacgcgcatcttctatttttatgacgacggcgcagaacacatttacctgtcgagcgcagactggatgtatcgcaatttcttccgccgcatcgaagtttgcttcccgctactggatgccaaggtaaagaagcgcgtgttcaaggaaggcctggaaccctatctcaaggataacagcaacgcctgggaaatgcagtccgatggccattacgaacgcaaggccagccgccgggccagttttgcagcacagcaattcctgatggcggagcatggacaggaaatattgcccgagagctga

SEQ ID NO: 158 - protein, 393 aa, Methylobacillus glycogenes
NLVRLMQIPDSVDRPDLKYPHYTASVPKELGKDADIFKAIRKQDILLHHPFQSFNPVIEFIKQAAEDPQVLAIKQTFYRTSADSTLMKSLIEAAQRGKEVTVVVELLARFDEEANINWAAQLENAGAHVVYGVVGHKTHAKMAMVVRRDEDKLRRYVHIATGNYHQRTARLYTDFGLLTCQEEISEDVNDVFAQLTGLGRASKLRHLWQSPFTLHQRLIKAIQHEAEIAKSGKKARIIAKMNALLDPDVIRALYDASNAGVQIELIVRGVCALRPGIPGISENIKVRSIVGRFLEHTRIFYFYDNGAEHIYLSSADWMYRNFFRRIEVCFPLLDAKVKKRVFKEGLEPYLKDNINAWEMLSDGSYESKPSRRAAYSAQQALMTELGQEVLPEI

SEQ ID NO: 159 - DNA, 1182 bp, Methylobacillus glycogenes
aatctggtacgcctgatgcagatccccgatagcgtggaccgcccagacctcaagtacccgcactacaccgccagcgtgcccaaggaactgggcaaggatgccgatatcttcaaggccatacgcaagcaggatattctgctgcatcacccctttcagtcatttaatccggtgattgaattcatcaagcaggcggcggaagatccgcaggtgctggcgatcaagcagaccttctaccgcaccagtgctgactccacgctgatgaaatccttgattgaagccgcgcagcgcggcaaggaagtcaccgtggtggttgagctgctggcgcgctttgatgaagaagccaatatcaattgggccgcccagctagagaatgccggagcccatgtggtgtacggtgtggtgggtcacaagacccacgccaagatggccatggtagtacgccgcgatgaagataagctgcgacgctatgtgcatattgcaactggcaattaccaccagcgtaccgcgcgcctctacaccgactttggcctattgacctgccaggaagaaatcagcgaagacgtcaatgacgtgtttgcacagctgactggcctgggtcgcgccagcaagctgcgtcacctctggcaatcgccctttaccttgcatcaacgcttgattaaggccattcagcatgaggccgagattgccaaatctggcaagaaggcgcgcattatcgccaagatgaatgcgctgctggacccggatgtgatacgtgcgctatacgatgcctccaatgccggggtacagatagagttgatcgtgcgcggggtctgcgccttgcgccctggcattcccggcatttccgagaatatcaaggttcgctcaattgttgggcgcttccttgagcacacacgcattttctatttctacgacaatggagccgagcatatctacctgtcgagtgcggattggatgtaccgcaacttcttccgccgcattgaagtttgcttcccgctgctggatgccaaggtgaaaaagcgcgtgttcaaggaagggctggagccttacctcaaggacaatatcaatgcatgggaaatgttgtcggatggcagctatgaatccaagcccagccgtcgtgcggcttactctgcgcaacaggcgctgatgacagaacttgggcaggaagtattgcccgagatttga

SEQ ID NO: 160 - protein, 693 aa, Methylobacillus rhizosphaerae
MLPVKLNPEYFINRELGILAFNRRVLAQAEDERVPLLERLKFLCIFSSNMDEFFEVRVAGLKNQIKYNSPHIGPDGLLPKQALATVSSMAHEMVELQYKILNDVVLPQLAAEEIRFIRRGDWNDTQREWIAAYFFRELMPILTPIGLDPAHPFPRVLNKSLNFAVELEGKDAFGRNSGVAIVQAPRALPRVIRLPREIAGCDHGFVFLSSILHAHVSELFSGMTVKGCYQFRVTRDTDLILDDEDTTDLRLALQGELAHRQYGDAVRLEVADNCPAEMSSFLLGQFGLTQEDLYQVNGLVNLVRLMQIPDSVDRPDLKFAHYTPSLPKELLKEADIFKAIRKQDILLHHPFQSFNPVIEFIKQAAEDPQVLAIKQTFYRTSADSTLMKSLIEAAQRGKEVTVVVELLARFDEEANINWAAKLENAGAHVVYGVVGHKTHAKMAMVVRREEDKLRRYVHIATGNYHQRTARLYTDFGVLTCQEEISEDVNDVFAQLTGLGRASKLRHLWQSPFTLHQRMVKAIQNEADIARSGKKARIIAKMNALLDPDVIRALYDASTAGVQIDLIVRGVCALRPGIPGVSENIRVRSIVGRFLEHTRIFYFYDNGAEHIHLSSADWMYRNFFRRIEICFPLLDAKAKRRVFKEGLEPYLKDNTNAWEMQQDGSYALKPNRRASFTAQQFLMQEHGQEILPDV

SEQ ID NO: 161 - DNA, 2082 bp, Methylobacillus rhizosphaerae
atgttgcccgttaaattgaatcccgaatactttatcaatcgcgaactcggcattctagccttcaatcgccgcgtgctggcgcaagcagaggatgaacgggttcccctattggaacgcctgaagtttctctgcattttcagcagcaacatggatgagtttttcgaggtgcgcgttgccggtctcaaaaaccagatcaagtacaactctccacacataggcccagatggcctcctgcccaagcaggcactggcaacagtcagcagcatggcgcacgagatggtcgagctccagtacaaaatcctcaacgatgtggtgctgccgcaactggcggcagaagaaatccgctttatccgccgtggggactggaacgatactcagcgcgaatggattgccgcctattttttccgcgagctgatgcctatcctcacgcctatcggcctggacccagcacatccatttccgcgcgtactcaacaagagcctcaatttcgccgttgaactggaaggcaaggatgctttcgggcgtaattccggcgtagccattgtgcaggcacctcgcgccttaccgcgcgtcatccgcctgccacgcgagattgccggctgtgaccatggttttgtattcctgtcctccatcctgcatgcccatgtcagcgaattattctccggcatgacggtgaagggttgctaccaattccgtgtcacgcgcgacactgacctgattctggatgatgaagacaccaccgacctcaggttggctttgcagggtgaactggctcatcgccagtacggcgacgcggtacgcctggaagtagcagataactgcccggcagagatgtcctccttcctgctcggccaatttgggttgacacaggaagacctgtatcaagtaaacggcctggtcaacctggtacgcctgatgcagattccggacagcgttgaccgccctgacctcaagtttgcacactacacaccgagtctgccgaaagaactgctcaaggaagcggatatcttcaaggcaatccgcaaacaggatattctgctgcatcatccgttccagtcattcaatcctgtgattgaattcatcaaacaggcggcagaagaccctcaggttctggcaatcaagcagacgttctatcgtaccagcgcagactcaacgctgatgaaatcattgattgaagcagcgcagcgcggcaaagaagtcacagtggtggtggaactgctggcgcgcttcgatgaagaagccaatattaattgggccgccaagcttgagaatgccggtgcccatgtagtctacggtgtcgtcggccacaagacacacgccaagatggccatggtcgtgcgccgcgaagaagataagctgcgtcgctatgtacatatcgccacaggcaattaccaccagcggacagcacggctgtataccgatttcggggtactgacctgccaggaggagatcagtgaggacgtcaatgatgtattcgcgcagctgaccggacttggccgcgccagcaaactgcgccatctctggcaatccccgttcaccttgcatcaacgcatggtcaaggccattcagaatgaagctgacattgcccgctccggcaaaaaagcccgtattatcgccaagatgaatgcgctgctggatcctgacgtgatccgtgccctttacgatgcatccacggccggtgtgcaaatcgacctcatcgtgcgtggcgtctgtgcattgcgccccggcattcccggcgtctcggaaaatatcagggtgcgctccatcgtcggccgttttctcgagcacacccgcattttctatttctatgacaatggggcagaacacatccatctttccagtgcagactggatgtaccgcaactttttccgccgtatcgagatctgcttcccgctactggatgcgaaagcgaagcgacgtgtattcaaggaagggctggaaccttaccttaaggacaataccaacgcctgggagatgcagcaggatggcagttatgcgctcaagccaaaccgcagggccagtttcactgcacagcagttcctgatgcaggaacatggacaggaaatattgccggacgtttga

SEQ ID NO: 162 - protein, 729 aa, Methylobacterium organophilum
APAEPSVGAARESVLEAGRSLRHTPERFVNRELSWLQFNRRVLEEASNPNHPLLERLRFLSISANNLDEFFMVRVAGLIDQVRAGITVPSQDGLSPSEQLVRIGAEVSRLAADQQARWRELREELHAADIDIVEPAALTAEQAAWLEEYFLNHVFPVLTPLAIDPAHPFPFIPNLGTTIALMLVRPKDGRLLRALIRLPGVIDRFVRLPVTESETAARLMPIEQVIGMFTGRLFPGYLVKGSGAFRVVRDSDLEIEEEAEDLVLHFETALKQRRRGVVIRLEVEAGMSEDLRSFVADELEIAADAIFLVEGMLALNELSQVVGIDRPDLKFKPYNPRFPERIRESGGDVFAAIRQKDFIVHHPYESFDSVVQFLAQAARDPNVVAIKQTLYRTSSNSPIVAALAEAAELGKSVTALVELKARFDEEANIRWARNLEKAGAQVVFGFVELKTHAKLSLVVRREGDKLVTYCHVGTGNYHPITARIYTDLSFFTADPAIARDVSRIFNFITGYAEPAELERMAVSPLTLKNRLLEHIEAEVAHAKAGRPAAIWIKCNSLVDGQIIDALYDASGAGVQIDCVVRGICCLRPGIPGLSETIRVKSIVGRFLEHGRIYAFGNGVGLPHPKATVYISSADLMSRNLDRRVEALLPITNPTVHQQVLDQIMLANLLDNRQSWRLLASGGCERIQPAEGEEPFNAHKYFMTNPSLSGRGKASKKSSPRALSRRAQRS

SEQ ID NO: 163 - DNA, 2190 bp, Methylobacterium organophilum
tcagctgcgttgcgcgcgtcggctgagggcccgcgggctcgacttcttcgaggccttgccgcgtcccgagaggctgggattggtcatgaaatacttgtgggcattgaacggctcctcgccctcggcgggctggatccgttcgcagccgcccgaggcgaggagccgccagctctgacggttgtcgagaaggttggccagcatgatctggtcgagcacctgctgatgcaccgtcgggttcgtgatcggcagcagcgcctcgacacggcggtcgaggttccggctcatcaggtcggccgaggagatgtagaccgtggccttggggtgcggcagcccgacgccgttgccgaaggcgtagatgcgcccgtgctcgaggaagcgcccgacgatcgacttcacccggatcgtctccgacaggccggggatgcccgggcgcaggcagcagatgccccggaccacgcagtcgatctgaacgccggctcccgaggcgtcgtagagcgcgtcgatgatctggccgtcgaccagggagttgcacttgatccagatcgcggccgggcgcccggccttcgcgtgggccacctccgcctcgatatgctccaggaggcggttcttcagcgtcagcggcgagaccgccatgcgctccagttcggccggctcggcgtagccggtgatgaagttgaagatgcgcgacacgtcccgcgcgatcgcgggatccgccgtgaagaacgacaggtccgtgtagatgcgcgcggtgatcgggtggtagttgccggtgccgacgtggcagtaggtgacgagcttgtcgccctcccgtcggaccaccagcgacagcttggcgtgcgtcttgagctcgacgaagccgaacacgacctgcgcgcccgccttctcgagattgcgcgcccagcggatgttggcttcctcgtcgaaccgcgccttcagctccacgagggcggtcacggacttgccgagctcggcggcctccgcgagggccgcgacgatcggagagttcgacgaggtgcggtagagcgtctgcttgatcgcgacgacgttcgggtcgcgcgcggcctgggcgaggaactgcaccaccgagtcgaaggattcgtaggggtggtggacgatgaagtccttctggcggatcgccgcgaagacgtcgccgccgctctcgcggatgcgctcggggaagcgcgggttgtagggcttgaacttcaggtcgggcctgtcgatgccgacgacctgggacagctcgttcagggccagcatgccctccacgaggaagatcgcgtccgcggcgatctcgagctcgtcggcgacgaagctgcgcagatcctccgacatgcccgcctcgacctcgaggcggatcacgacgccgcggcggcgctgcttcaacgcggtctcgaaatgcaggacgaggtcttcggcctcctcctcgatctccaggtcggagtcgcggaccacgcggaacgcgccgctgcccttcacgaggtagcccgggaagagccggccggtgaacatcccgatcacctgctcgatcggcatcagccgcgccgcggtctcgctctcggtcaccggcaggcgcacgaagcggtcgatgacgccgggcaggcggatgagcgcgcgcagcagccttccgtccttcggccgaacaagcatcagcgcgatggtggtgccgagattcgggatgaacgggaacgggtgagccggatcgatcgccagcggcgtcaggaccgggaagacgtggttgaggaagtactcctccagccacgccgcctgctcggccgtgagggcggcgggctcgacgatgtcgatgtcggccgcgtgcagctcctcgcgcagctcccgccagcgggcctgctggtcggcggcgaggcgcgagacctcggcgccgatccggaccagctgctccgatggcgacaggccgtcctgcgacggcaccgtgatcccggcccggacctgatcgatcaggccggcgacgcggaccatgaagaattcgtcgaggttgttggccgagatcgacaggaagcggaggcgctccaggagcgggtggttcggattcgacgcctcctccagcacgcgccgattgaactgaagccaggacagctcgcggttcacgaaccgctccggcgtgtgacgcagggaccgccccgcttccagaaccgactcacgggccgccccgaccgacggctccgccggggc

SEQ ID NO: 164 - protein, 788 aa, Methylorubrum extorquens
MSEVESDVVARDTEATETEETSLATERGVRSESARARTARAARILAAEKAAEKPSEADAKVESDAAEAAREPVLEAGRSLRHSPERFVNRELSWLQFNRRVLEESANPNHPLLEQLRFLSISANNLDEFFMVRVAGLHDQVRAGLVVPSQDGLTPSEQLARIGTEVSRLALDQQDRWRALREELNGNGIHLAEPAELSAEHLAWLDDYFLTYIFPVLTPLAIDPAHPFPFIPNLGFTVALMMVRPRDGRTLRALIRLPSLLDRFVRLPDVAGDGTARFIAIEQVIAKYASRLFPGYSLKGQGAFRVVRDSDLEIEEEAEDLVLHFESAIKRRRRGVVIRLEVEAGMTEELRSFVADELEIAPDSVFVVEGMLALNELSQIVGIDRPDLKFKPYNPRFPERIRESGGDVFAAIRQKDFIVHHPYESFDSVVQFLAQAARDPNVVAIKQTLYRTSSNSPIVAALAEAAEAGKSVTALVELKARFDEEANIRWARNLEKAGAQVVFGFVELKTHAKLSMVVRREGDRLVTYCHVGTGNYHPITARIYTDLSFFTADPAIARDVSRIFNFITGYAEPAELERMAVSPLTLKPRLLQHIEEEIAHAKAGRPAAIWIKCNSLVDSQIIDALYDASQEGVQIDCIVRGICCLRPGIPGLSDTIRVKSIVGRFLEHERVYAFGNGAGLPHPKATLYISSADLMQRNLDRRVESLLPITNPTVHQQVLDQIMLANLLDNRQSWRVLASGASERISPADGEEPFNAHKYFMTNPSLSGRGKSSKKSSPRALSRRAQRS

SEQ ID NO: 165 - DNA, 2367 bp, Methylorubrum extorquens
ttgtcggaagtggagtcggatgtcgtcgcccgggatacggaggcgaccgagaccgaagagaccagcctcgccaccgagcggggtgtgcgcagcgaatccgcccgcgcccggacggcccgcgccgcccgcatcctcgcggcggagaaggccgccgagaagccgtcggaggcggatgccaaggtggagagcgatgcggccgaggccgcccgcgagccggtgctggaggctgggcgatcgctccgccactcgcccgagcggttcgtgaaccgtgagctgtcctggctccagttcaaccgccgggttctggaggaatcggccaaccccaaccatccgctgctggagcagctccgcttcctctcgatctcggccaacaatctggacgagttcttcatggtgcgtgtcgccggcctgcacgatcaggtccgcgccggcctcgtcgtgccctcgcaggacggcctgaccccctccgagcagcttgcccgcatcggcacggaagtctcgcggctggcgctggaccagcaggatcgctggcgcgcgctgcgcgaggagctaaacggcaacggtattcacctcgcggagccggcggagctgtcggcggagcaccttgcttggctcgacgactatttcctcacctacatcttcccggtgctgacgccgctggcgatcgatccggcccacccgttcccgttcatccccaatctcggcttcaccgtcgcgctgatgatggtgcggccccgtgacgggcgcaccctgcgcgccctgatccgcctgccgtcgctgctcgaccggttcgtgcgcctgcccgacgtggccggcgacggcactgcccgcttcatcgccatcgagcaggtgatcgcgaaatacgcgagccggctcttccccggctactcactgaaggggcagggcgccttccgcgtcgtgcgcgattccgatctcgagatcgaggaggaggcggaagacctcgtcctgcacttcgaatcggcgatcaagcgccgccgccgcggcgtcgtcatccgcctggaggtcgaggcgggcatgacggaggagctgcgctccttcgttgccgacgaattggagatcgcccccgattcggtcttcgtggtcgaggggatgctggcgctcaacgagctgtcgcagatcgtcgggattgaccgaccggacctcaagttcaagccctacaacccgcgcttccccgagcgcatccgtgaatcgggcggcgacgtcttcgcggcgatccgccagaaggatttcatcgtccaccatccctacgagtcgttcgactcggtggtgcagttcctggcccaggccgcccgcgatccgaacgtggtggcgatcaagcagacgctctaccgcacctcatcgaactcgccgatcgtggccgcgctcgcggaggcggcggaggccggcaagtccgtcaccgcactggtcgagctgaaggcccggttcgacgaggaggccaatatccgctgggcgcgcaacctcgagaaggcgggcgcgcaggtggtgttcggcttcgtcgagctgaagactcacgccaagctgtcgatggtggtgcgccgcgagggcgaccgcctcgtcacctactgccatgtcggcaccggcaactatcacccgatcaccgcgcgcatctacaccgacctgtccttcttcaccgccgacccggccatcgcccgggacgtctcgcgcatcttcaacttcatcaccggctacgccgagccggcggagctggagcgcatggcggtgtcgccgctgaccctgaagccgcgcctcttgcagcacatcgaggaggagatcgcccacgccaaggccgggcgcccggcggcgatctggatcaagtgcaactcgctggtcgacagccagatcatcgatgcgctctacgatgccagccaggagggcgtgcagatcgactgcatcgtgcgcggcatctgctgcctgcggccgggcattccgggcctgtccgacacgatccgggtcaagtcgatcgtcgggcgcttcctcgagcacgagcgcgtctacgccttcggcaacggcgccgggctgccgcacccgaaggccaccctctacatttcctcggccgacctgatgcagcgcaacctcgatcgacgcgtcgaatccctgctgccgatcaccaatccgactgtgcatcagcaggtgctcgatcagatcatgctggcaaaccttctcgacaaccgacagagctggcgtgtactggcatcgggtgcgagcgagcggatcagccctgcggacggggaggaaccgttcaatgcgcacaagtatttcatgacgaatccaagcctgtccgggcgcggcaagtcgtcgaagaagtcgagcccgcgggcgctcagccgtcgcgcccagcggtcctga

SEQ ID NO: 166 - protein, 688 aa, Escherichia coli
MGQEKLYIEKELSWLSFNERVLQEAADKSNPLIERMRFLGIYSNNLDEFYKVRFAELKRRIIISEEQGSNSHSRHLLGKIQSRVLKADQEFDGLYNELLLEMARNQIFLINERQLSVNQQNWLRHYFKQYLRQHITPILINPDTDLVQFLKDDYTYLAVEIIRGDTIRYALLEIPSDKVPRFVNLPPEAPRRRKPMILLDNILRYCLDDIFKGFFDYDALNAYSMKMTRDAEYDLVHEMEASLMELMSSSLKQRLTAEPVRFVYQRDMPNALVEVLREKLTISRYDSIVPGGRYHNFKDFINFPNVGKANLVNKPLPRLRHIWFDKAQFRNGFDAIRERDVLLYYPYHTFEHVLELLRQASFDPSVLAIKINIYRVAKDSRIIDSMIHAAHNGKKVTVVVELQARFDEEANIHWAKRLTEAGVHVIFSAPGLKIHAKLFLISRKENGEVVRYAHIGTGNFNEKTARLYTDYSLLTADARITNEVRRVFNFIENPYRPVTFDYLMVSPQNSRRLLYEMVDREIANAQQGLPSGITLKLNNLVDKGLVDRLYAASSSGVPVNLLVRGMCSLIPNLEGISDNIRAISIVDRYLEHDRVYIFENGGDKKVYLSSADWMTRNIDYRIEVATPLLDPRLKQRVLDIIDILFSDTVKARYIDKELSNRYVPRGNRRKVRAQLAIYDYIKSLEQPE

SEQ ID NO: 167 - DNA, 2067 bp, Escherichia coli
atgggtcaggaaaagctatacatcgaaaaagagctcagttggttatcgttcaatgaacgcgtgcttcaggaagcggcggacaaatctaacccgctgattgaaaggatgcgtttcctggggatctattccaataaccttgatgagttctataaagtccgcttcgctgaactgaagcgacgcatcattattagcgaagaacaaggctccaactctcattcccgccatttactgggcaaaattcagtcccgggtgctgaaagccgatcaggaattcgacggcctctacaacgagctattgctggagatggcgcgcaaccagatcttcctgattaatgaacgccagctctccgtcaatcaacaaaactggctgcgtcattattttaagcagtatctgcgtcagcacattacgccgattttaatcaatcctgacactgacttagtgcagttcctgaaagatgattacacctatctggcggtggaaattatccgtggcgataccatccgttacgcgctgctggagatcccatcagataaagtgccgcgctttgtgaatttaccgccagaagcgccgcgtcgacgcaagccgatgattcttctggataacattctgcgttactgccttgatgatattttcaaaggcttctttgattatgacgcgctgaatgcctattcaatgaagatgacccgcgatgccgaatacgatttagtgcatgagatggaagccagcctgatggagttgatgtcttccagtctcaagcagcgtttaactgctgagccggtgcgttttgtttatcagcgcgatatgcccaatgcgctggttgaagtgttacgcgaaaaactgactatttcccgctacgactccatcgtccccggcggtcgttatcataattttaaagactttattaatttccccaatgtcggcaaagccaatctggtgaacaaaccactgccgcgtttacgccatatttggtttgataaagcccagttccgcaatggttttgatgccattcgcgaacgcgatgtgttgctctattatccttatcacacctttgagcatgtgctggaactgctgcgtcaggcttcgttcgacccgagcgtactggcgattaaaattaacatttaccgcgtggcgaaagattcacgcatcatcgactcgatgatccacgccgcacataacggtaagaaagtcaccgtggtggttgagttacaggcgcgtttcgacgaagaagccaacattcactgggcgaagcgcctgaccgaagcaggcgtgcacgttatcttctctgcgccggggctgaaaattcacgccaaactgttcctgatttcacgtaaagaaaacggtgaagtggtgcgttatgcacacatcgggaccgggaactttaacgaaaaaaccgcgcgtctttatactgactattcgttgctgaccgccgatgcgcgcatcaccaacgaagtacggcgggtatttaactttattgaaaacccataccgtccggtgacatttgattatttaatggtatcgccgcaaaactcccgccgcctattgtatgaaatggtggaccgcgagatcgccaacgcgcagcaagggctgcccagtggtatcaccctgaagctaaataaccttgtcgataaaggcctggttgatcgtctgtatgcggcctccagctccggcgtaccggttaatctgctggttcgcggaatgtgttcgctgatccccaatctggaaggcattagcgacaacattcgtgccatcagtattgttgaccgttaccttgaacatgaccgggtttatatttttgaaaatggcggcgataaaaaggtctacctttcttccgccgactggatgacgcgcaatattgattatcgtattgaagtggcgacgccgctgctcgatccgcgcctgaagcagcgggtactggacatcatcgacatattgttcagcgatacggtcaaagcacgttatatcgataaagaactcagtaatcgctacgttccccgcggcaatcgccgcaaagtacgggcgcagttggcgatttatgactacatcaaatcactcgaacaacctgaataa

SEQ ID NO: 168 - protein, 249 aa, Methylobacillus flagellatus
MLDRQSSLGTRPGVHQLYVSLARNASEIAEAQRLRYKVFAEEMGANVSGTEGLDQDGFDAFCDHLLVRNHETGEVVGTYRILSPAMANEAGGYYSAGEFDLSRLRHLAPSMVEVGRACVHKDYRLGGTITLLWAGLANYMKVHRYEYMIGCGSIGMADGGHMAASLYHQLKQDHLSPVEYRVFPNCPLPLEALRNDLEVACPPLIKGYLRLGAYICGAPAWDPDFNTADMLVMLPLSRLNKRYAAHFFK

SEQ ID NO: 169 - DNA, 750 bp, Methylobacillus flagellatus
atgcttgaccggcagtcttccctcggcaccaggcccggtgtccaccagctctatgtcagccttgcacgcaacgcatccgaaatcgccgaggcacaacgcctgcgctacaaagtatttgcagaggagatgggcgccaacgtctccggcactgaaggactggaccaagatggctttgacgccttttgcgatcacttgctggtccgcaaccatgaaacaggcgaagtcgtcggcacttaccgcatattgagtccggccatggccaacgaagctggcggctactactccgctggcgaattcgacctctcgcgcctgcgccatcttgcccccagcatggtggaagttggccgcgcctgcgtacacaaggattaccgcctgggcggcacgatcaccctgctctgggccgggctggccaactacatgaaagtgcatcgctacgagtacatgatcggctgtggcagcatcggcatggcagacggcggccatatggcggctagcttgtatcaccagctaaaacaggatcacctttcgccagtggaataccgcgtattccccaattgcccgctgccgctggaagccttgcgcaacgacctggaagtcgcttgcccgcccctgatcaaaggttacctgcgcctgggcgcatatatctgcggcgcaccagcttgggaccctgatttcaatacagcagacatgctggtcatgctaccattgtcgcgactcaacaaacgttatgcagctcactttttcaaataa

SEQ ID NO: 170 - protein, 248 aa, Methylobacillus flagellatus
MLERRLSPKAAEDDAPLHISFARNPSEVAEAQRLRYRIFVEEMGANLPSKDGYDRDGFDAFCDHLLVRNNNGEVVGTYRILSPFMANEAGGYYSAAEFDLSRLSPLFDRTVEVGRACVHEDYRHGGTITMLWAGLAKYMQANRYEYMIGCGSVGMGDGGHMAASLYNRLREDYLSPAEYRVFPRVPLPLDALRSDMPATIPPLMKGYLRLGAYICGEPAWDPDFNTADMLVMLPLSRLNKRYAAHFFK

SEQ ID NO: 171 - DNA, 747 bp, Methylobacillus flagellatus
atgctggaacggcgtttatcacccaaggcagcggaggacgatgctccgctgcacatcagctttgcccgcaacccgtctgaagtcgctgaagcgcagcgcctgcgctaccgtatctttgttgaagaaatgggtgccaacttgcccagcaaggacggctacgaccgtgacggctttgacgctttctgcgaccacctgctggtacgcaacaacaacggcgaagtggtcggcacctatcgcatattgagcccattcatggccaatgaagccggtggctattactcggcggccgagttcgacctgagccgtttgagcccactgttcgaccgtactgtagaagtcggccgtgcctgcgtgcatgaggattatcgccatggcggcaccatcaccatgttgtgggctggcttggccaaatacatgcaagccaaccgttatgaatacatgataggttgcggcagcgtaggcatgggtgacggtggacacatggcagccagtctttataatagattgcgtgaagactatttgtcgcccgctgaataccgcgtgtttccacgtgttccgctgccactggatgcgttgcgcagcgacatgccagccaccatcccgccattgatgaaaggctacctgcgactgggtgcttatatctgtggcgaaccggcctgggatcctgacttcaacaccgctgacatgctggtgatgttgccgctgtcgcgtttgaacaaacgttacgcagcgcactttttcaaataa

SEQ ID NO: 172 - protein, 249 aa, Methylobacillus glycogenes
MLDRQLPLGNKPGASQLYVSLARNASEIAEAQRLRYKVFAEEMGANLAGANGLDQDGFDAFCDHLLVRNQDTGEVVGTYRILSPAMANEAGGYYSAAEFDLTRLRHLAPSMVEVGRACVHKDYRMGGTITLLWAGLANYMKVHRYEYMIGCGSIGMADGGHMAASLYHQLQKEHLSPAEYRVFPNCPLPLEALRHDQEVTCPPLIKGYLRLGAYICGAPAWDPDFNTADILVMLPLARLNKRYAAHFFK

SEQ ID NO: 173 - DNA, 750 bp, Methylobacillus glycogenes
atgcttgatcggcagttacccctaggcaacaaacccggagcgagccaactttacgtcagcctggcccgcaacgcctctgaaattgcagaagcgcagcgcctgcgttacaaagtatttgcagaagaaatgggtgccaatctggctggtgcgaatggcctggatcaagatggctttgatgcattttgcgaccacttgctggtgcgcaatcaagacacgggggaagtggtaggcacttaccgcatattaagccccgccatggccaatgaagcaggcggttattattccgccgctgaatttgacctcacgcgtttacgtcacctggcacccagcatggtagaagtgggccgtgcctgcgtgcacaaggattaccgcatgggcggcaccattactttgttgtgggcaggtctcgccaactacatgaaagtacacagatacgaatacatgataggttgcggcagcataggcatggccgatggcggtcatatggcagcaagcctgtatcaccagttgcagaaagagcacctgtcgcctgctgaataccgtgtgttccccaattgccccttgccgctggaagccctgcgtcacgaccaagaagtgacttgcccgccattgatcaaaggctatttgcgcctgggtgcctatatttgcggcgcacccgcctgggaccctgatttcaatacggccgatatcctggtcatgctaccattagcccgactcaacaaacgctatgcagctcactttttcaaatag

SEQ ID NO: 174 - protein, 249 aa, Methylobacillus rhizosphaerae
MLDRQSSLGIKAGASQLHVSLARNPSEIAEAQRLRYKIFAEEMGANLSSSDGLDQDGFDEFCDHLLVRNHETGEVVGTYRILSPAMANEAGGYYSSGEFDLSRLRHLASSMVEVGRACVHKDYRLGGTITLLWAGLANYMKVHRYEYMIGCGSIGMADGGHMAASLYQQLQNDHLSPPEYRVFPNCPLPLEALRHDLEVNCPPLIKGYLRLGAYICGAPAWDPDFNTADILVMLPLSRLNKRYAAHFFK

SEQ ID NO: 175 - DNA, 750 bp, Methylobacillus rhizosphaerae
atgctcgatcggcagtcttcccttggcatcaaggccggggccagccaattgcatgtcagtcttgcccgcaacccttccgaaattgcagaagcccaacgtttacgttacaaaatatttgctgaagaaatgggagccaatctttccagctccgatggcctggatcaggatggttttgatgagttctgcgaccacttgctggttcgcaatcatgaaaccggcgaagtagtcggcacctaccgcatcctcagcccggccatggccaatgaagctggtggctattactcatccggtgaattcgacttgtcgcgactgcgccaccttgcctcaagcatggtggaagtaggtcgtgcctgcgtgcacaaggattatcgactgggcggcaccattaccctgctgtgggcaggcctggccaattacatgaaggtacatcgctatgagtacatgataggctgcggcagtattggcatggccgatggcggccacatggcggccagcctgtatcagcaattacaaaacgaccacctatccccaccggaatatcgtgtatttcccaattgccccctgccactggaagcattgcgccatgacctcgaggtgaattgcccgccgctgatcaaaggctacttgcgtctgggtgcctatatttgcggcgctcctgcctgggaccctgatttcaacaccgcagatattctggtcatgctaccattgtcgagactcaacaaacgctatgcagctcattttttcaagtaa

SEQ ID NO: 176 - protein, 332 aa, Methylobacterium organophilum
MVANLARGAYSALGAGWHKGVQWGVGAPIAKLRRRAVPLPGVAGAGGIDDVLSAERAIRLPEPFEGRSLGRIGSLEVRLATRKSEIRRAQRLRYKVFYEEMSAVPSGLAALSRRDVDGYDAVCDHLLVLDHAAPRRKKPFVEPRPKVVGTYRLLRGEVAERHTGFYSESEYDLAPLLAAQGHRRLLELGRSCVLKPYRSKRTVELLWQGIYAYVLHHRIDALIGCASLEGTDPDRLALPLAFLHHHARAPEGWRARALPERAVAMDRMPREAVDAKAALQALPPLIKGYLRLGATFGDGAVIDRQFGTTDVFVTLPVEVIGARYRGHFAPAG

SEQ ID NO: 177 - DNA, 999 bp, Methylobacterium organophilum
atggtcgccaatctcgcccgcggagcctacagcgcgctcggagccggctggcacaagggcgtgcaatggggcgtcggcgcgccgatcgccaagctgcgccgccgggcagtcccgctgccgggcgtcgcgggcgcgggcggaatcgacgacgtgctctcggccgagcgggcgatccgcctgcccgagccgttcgagggccgcagcctcggccgcatcggcagcctcgaggtccggctggcgacgcggaagtccgagattcggcgggcccagcggctgcgctacaaggtcttctacgaggagatgtcggcggtgccctccgggctcgccgcgctgtcccgccgcgacgtcgacggctacgacgcggtctgcgaccacctgctcgttctcgaccacgcggcgccgaggcggaagaagccgttcgtcgagccgcgcccgaaggtcgtcggcacctaccggctgctgcgcggcgaggtcgccgagcggcacaccggcttctattccgagagcgagtacgacctcgcgccgctgctcgccgcgcaggggcaccggcggctcctggaactcggccgctcctgcgtgctcaagccctaccggagcaagcggaccgtcgagctgctgtggcaggggatctacgcctacgtcctgcaccaccggatcgacgcgctgatcggctgcgcgagcctggagggtaccgatccggaccggctggccctgccgctcgccttcctgcaccaccatgcccgcgcgccggagggctggcgggcccgggcgctgccggagcgggcggtggcgatggaccggatgccgcgcgaggcggtggatgccaaggccgccctgcaggcgctgccgccgctgatcaagggctacctgcgcctcggcgcgaccttcggcgacggcgcggtgatcgaccgccagttcggcacgacggacgtgttcgtcacgctgccggtcgaggtgatcggcgcgcgctaccggggccatttcgcgccggcggggtga

SEQ ID NO: 178 - protein, 332 aa, Methylorubrum extorquens
MLPNFSPREATAAWKAGWETKVQAPFARFRQTFEGGDLALPGGAPILLKNRAKRPLLEPGLDPSLGRIGALEVRLATTKSEIRRAQRLRYRVFYEEMSAVPTGMAALKRRDVDAYDAICDHLLVIDHAATDAKPFRKARPKVVGTYRLLRQDRAEAHFGFYSSGEYDLAPLLERHPGKRFLELGRSCVLKPYRTKRTVELLWHGIWAYVQHHRIDAMLGCASLEGTDPERLALPLSFLHHHARAPEAWRARALPERYVAMDRLAKEAVDPKAALMALPPLVKGYLRVGATFGDGAVVDRQFGTTDVLVVLPVSGIAARYIGHFGASADRHAA

SEQ ID NO: 179 - DNA, 999 bp, Methylorubrum extorquens
atgctgccgaatttttccccgcgcgaggccacggccgcgtggaaggccggctgggagaccaaggttcaggcgcccttcgcccgcttccgccagaccttcgagggcggcgacctcgccctgcccggcggtgcgccgatccttctgaagaaccgggccaagcgcccgctgctcgaaccggggctcgaccccagcctcggtcggatcggggcgctcgaagtgcggctcgccaccaccaagtccgagatccgccgggcgcagcgcctgcgctaccgcgtgttctacgaggagatgtcggcggtgccgaccggcatggccgcgctcaagcgccgcgatgtcgatgcctacgacgcgatctgcgaccacctcctcgtcatcgaccacgcggcgaccgacgcgaagcccttccgcaaggcccggccgaaggtggtcggcacctaccggctgctgcgccaggaccgggcggaggcgcatttcggcttctactcctcgggcgagtacgacctcgcgccgctgctggagcgccatccaggcaagcgcttcctcgaactcgggcgctcctgcgtgctgaagccgtaccgcaccaagcgcaccgtcgaactcctgtggcacggcatctgggcctatgtgcagcaccaccgcatcgacgcgatgctgggctgcgccagcctggagggcaccgatccggagcgtctggcgctgcccttgagctttcttcaccaccatgcccgcgcccccgaggcgtggcgggcccgcgccctgccggagcgctacgtcgcgatggaccggctggcgaaggaggcggtcgatccgaaggcggcgctgatggcgctgccgccgctggtgaagggctatctccgggtcggggcgaccttcggcgacggcgcggtggtggaccgccagttcggcaccaccgacgttctcgtggtgctgccggtctcaggcatcgccgcgcgctacatcggccatttcggcgcgagtgcggatcggcacgccgcctga

SEQ ID NO: 180 - protein, 352 aa, Methylorubrum extorquens
MLSPRKRTHRAASRDGIVSIMLPNFSPREATAAWKAGWETKVQAPFARFRQTFEGGDLALPGGAPILLKNRAKRPLLEPGLDPSLGRIGALEVRLASTKSEIRRAQRLRYRVFYEEMSAVPTGMAALKRRDVDAYDAICDHLLVIDHAATDAKPFRKARPKVVGTYRLLRQDRAEAHFGFYSSGEYDLAPLLERHPGKRFLELGRSCVLKPYRTKRTVELLWHGIWAYVQHHRIDAMLGCASLEGTDPERLALPLSFLHHHARAPEAWRARALPERYVAMDRLAKEAVEPKAALMALPPLVKGYLRVGATFGDGAVVDRQFGTTDVLVVLPVSGIAARYIGHFGAGADRHAA

SEQ ID NO: 181 - DNA, 1059 bp, Methylorubrum extorquens
atgttgtcgccgcgcaagaggacgcatcgcgcggcctcccgcgacgggatcgtgtcgatcatgctgccgaatttttccccgcgcgaggccacggccgcgtggaaggccggctgggagaccaaggttcaggcgcccttcgcccgcttccgccagaccttcgagggcggtgacctcgccctgcccggcggtgcgccgatccttctgaagaaccgggccaagcgcccgctgctcgaaccggggctcgaccccagcctcggccggatcggggcgctcgaagtgcggctcgcctccaccaagtccgagatccgccgggcgcagcgcctgcgctaccgcgtgttctacgaggagatgtcggcggtgccgaccggcatggccgctctcaagcgccgcgatgtcgatgcctacgacgcgatctgcgaccacctcctcgtcatcgaccacgcggccaccgacgcgaagcccttccgcaaggcccggccgaaggtggtcggcacctaccggctgttgcgccaggaccgggcggaggcgcatttcggcttctactcctcgggcgagtacgacctcgcgccgctgctggagcgccatccgggcaaacgcttcctcgaactcggccgctcctgcgtgctgaagccctaccgcaccaagcgcaccgtcgaactcctgtggcacggcatctgggcctatgtgcagcaccaccgcatcgacgcgatgctcggctgcgccagcctggagggcaccgatccggagcgtctggcgctgcccttgagcttcctccaccaccatgcccgcgcccccgaggcgtggcgggcccgcgccctgccggagcgctacgtcgcgatggaccggctggccaaggaggcggtcgaaccgaaggccgcgctgatggcgctaccgccgctggtgaagggttatctccgggtcggggcgaccttcggcgacggcgcggtggtggaccgccagttcggcaccaccgacgtgctcgtggtgctgccggtctcaggcatcgccgcgcgctacatcggccatttcggcgcgggtgcggatcggcacgccgcctga